European Patent Specification EP 3 972 610 B1, published September 3, 2025. Title: MINIGENE THERAPY. Applicant: University of Massachusetts. Application Not Yet Assigned. The sequence listing filed with the application follows.

SEQUENCE LISTING (39 sequences)

SEQ ID NO: 1 - protein, 2479 aa, Homo sapiens
MPPNINWKEIMKVDPDDLPRQEELADNLLISLSKVEVNELKSEKQENVIHLFRITQSLMKMKAQEVELALEEVEKAGEEQAKFENQLKTKVMKLENELEMAQQSAGGRDTRFLRNEICQLEKQLEQKDRELEDMEKELEKEKKVNEQLALRNEEAENENSKLRRENKRLKKKNEQLCQDIIDYQKQIDSQKETLLSRRGEDSDYRSQLSKKNYELIQYLDEIQTLTEANEKIEVQNQEMRKNLEESVQEMEKMTDEYNRMKAIVHQTDNVIDQLKKENDHYQLQVQELTDLLKSKNEEDDPIMVAVNAKVEEWKLILSSKDDEIIEYQQMLHNLREKLKNAQLDADKSNVMALQQGIQERDSQIKMLTEQVEQYTKEMEKNTCIIEDLKNELQRNKGASTLSQQTHMKIQSTLDILKEKTKEAERTAELAEADAREKDKELVEALKRLKDYESGVYGLEDAVVEIKNCKNQIKIRDREIEILTKEINKLELKISDFLDENEALRERVGLEPKTMIDLTEFRNSKHLKQQQYRAENQILLKEIESLEEERLDLKKKIRQMAQERGKRSATSGLTTEDLNLTENISQGDRISERKLDLLSLKNMSEAQSKNEFLSRELIEKERDLERSRTVIAKFQNKLKELVEENKQLEEGMKEILQAIKEMQKDPDVKGGETSLIIPSLERLVNAIESKNAEGIFDASLHLKAQVDQLTGRNEELRQELRESRKEAINYSQQLAKANLKIDHLEKETSLLRQSEGSNVVFKGIDLPDGIAPSSASIINSQNEYLIHLLQELENKEKKLKNLEDSLEDYNRKFAVIRHQQSLLYKEYLSEKETWKTESKTIKEEKRKLEDQVQQDAIKVKEYNNLLNALQMDSDEMKKILAENSRKITVLQVNEKSLIRQYTTLVELERQLRKENEKQKNELLSMEAEVCEKIGCLQRFKEMAIFKIAALQKVVDNSVSLSELELANKQYNELTAKYRDILQKDNMLVQRTSNLEHLECENISLKEQVESINKELEITKEKLHTIEQAWEQETKLGNESSMDKAKKSITNSDIVSISKKITMLEMKELNERQRAEHCQKMYEHLRTSLKQMEERNFELETKFAELTKINLDAQKVEQMLRDELADSVSKAVSDADRQRILELEKNEMELKVEVSKLREISDIARRQVEILNAQQQSRDKEVESLRMQLLDYQAQSDEKSLIAKLHQHNVSLQLSEATALGKLESITSKLQKMEAYNLRLEQKLDEKEQALYYARLEGRNRAKHLRQTIQSLRRQFSGALPLAQQEKFSKTMIQLQNDKLKIMQEMKNSQQEHRNMENKTLEMELKLKGLEELISTLKDTKGAQKVINWHMKIEELRLQELKLNRELVKDKEEIKYLNNIISEYERTISSLEEEIVQQNKFHEERQMAWDQREVDLERQLDIFDRQQNEILNAAQKFEEATGSIPDPSLPLPNQLEIALRKIKENIRIILETRATCKSLEEKLKEKESALRLAEQNILSRDKVINELRLRLPATAEREKLIAELGRKEMEPKSHHTLKIAHQTIANMQARLNQKEEVLKKYQRLLEKAREEQREIVKKHEEDLHILHHRLELQADSSLNKFKQTAWDLMKQSPTPVPTNKHFIRLAEMEQTVAEQDDSLSSLLVKLKKVSQDLERQREITELKVKEFENIKLQLQENHEDEVKKVKAEVEDLKYLLDQSQKESQCLKSELQAQKEANSRAPTTTMRNLVERLKSQLALKEKQQKALSRALLELRAEMTAAAEERIISATSQKEAHLNVQQIVDRHTRELKTQVEDLNENLLKLKEALKTSKNRENSLTDNLNDLNNELQKKQKAYNKILREKEEIDQENDELKRQIKRLTSGLQGKPLTDNKQSLIEELQRKVKKLENQLEGKVEEVDLKPMKEKNAKEELIRWEEGKKWQAKIEGIRNKLKEKEGEVFTLTKQLNTLKDLFAKADKEKLTLQRKLKTTGMTVDQVLGIRALESEKELEELKKRNLDLENDILYMRAHQALPRDSVVEDLHLQNRYLQEKLHALEKQFSKDTYSKPSISGIESDDHCQREQELQKENLKLSSENIELKFQLEQANKDLPRLKNQVRDLKEMCEFLKKEKAEVQRKLGHVRGSGRSGKTIPELEKTIGLMKKVVEKVQRENEQLKKASGILTSEKMANIEQENEKLKAELEKLKAHLGHQLSMHYESKTKGTEKIIAENERLRKELKKETDAAEKLRIAKNNLEILNEKMTVQLEETGKRLQFAESRGPQLEGADSKSWKSIVVTRMYETKLKELETDIAKKNQSITDLKQLVKEATEREQKVNKYNEDLEQQIKILKHVPEGAETEQGLKRELQVLRLANHQLDKEKAELIHQIEANKDQSGAESTIPDADQLKEKIKDLETQLKMSDLEKQHLKEEIKKLKKELENFDPSFFEEIEDLKYNYKEEVKKNILLEEKVKKLSEQLGVELTSPVAASEEFEDEEESPVNFPIY

SEQ ID NO: 2 - protein, 1116 aa, Homo sapiens
TENISQGDRISERKLDLLSLKNMSEAQSKNEFLSRELIEKERDLERSRTVIAKFQNKLKELVEENKQLEEGMKEILQAIKEMQKDPDVKGGETSLIIPSLERLVNAIESKNAEGIFDASLHLKAQVDQLTGRNEELRQELRESRKEAINYSQQLAKANLKIDHLEKETSLLRQSEGSNVVFKGIDLPDGIAPSSASIINSQNEYLIHLLQELENKEKKLKNLEDSLEDYNRKFAVIRHQQSLLYKEYLSEKETWKTESKTIKEEKRKLEDQVQQDAIKVKEYNNLLNALQMDSDEMKKILAENSRKITVLQVNEKSLIRQYTTLVELERQLRKENEKQKNELLSMEAEVCEKIGCLQRFKEMAIFKIAALQKVVDNSVSLSELELANKQYNELTAKYRDILQKDNMLVQRTSNLEHLECENISLKEQVESINKELEITKEKLHTIEQAWEQETKLGNESSMDKAKKSITNSDIVSISKKITMLEMKELNERQRAEHCQKMYEHLRTSLKQMEERNFELETKFAELTKINLDAQKVEQMLRDELADSVSKAVSDADRQRILELEKNEMELKVEVSKLREISDIARRQVEILNAQQQSRDKEVESLRMQLLDYQAQSDEKSLIAKLHQHNVSLQLSEATALGKLESITSKLQKMEAYNLRLEQKLDEKEQALYYARLEGRNRAKHLRQTIQSLRRQFSGALPLAQQEKFSKTMIQLQNDKLKIMQEMKNSQQEHRNMENKTLEMELKLKGLEELISTLKDTKGAQKVINWHMKIEELRLQELKLNRELVKDKEEIKYLNNIISEYERTISSLEEEIVQQNKFHEERQMAWDQREVDLERQLDIFDRQQNEILNAAQKFEEATGSIPDPSLPLPNQLEIALRKIKENIRIILETRATCKSLEEKLKEKESALRLAEQNILSRDKVINELRLRLPATAEREKLIAELGRKEMEPKSHHTLKIAHQTIANMQARLNQKEEVLKKYQRLLEKAREEQREIVKKHEEDLHILHHRLELQADSSLNKFKQTAWDLMKQSPTPVPTNKHFIRLAEMEQTVAEQDDSLSSLLVKLKKVSQDLERQREITELKVKEFENIKLQLQENHEDEVKKVKAEVEDLKYLLD

SEQ ID NO: 3 - protein, 601 aa, Homo sapiens
TENISQGDRISERKLDLLSLKNMSEAQSKNEFLSRELIEKERDLERSRTVIAKFQNKLKELVEENKQLEEGMKEILQAIKEMQKDPDVKGGETSLIIPSLERLVNAIESKNAEGIFDASLHLKAQVDQLTGRNEELRQELRESRKEAINYSQQLAKANLKIDHLEKETSLLRQSEGSNVVFKGIDLPDGIAPSSASIINSQNEYLIHLLQELENKEKKLKNLEDSLEDYNRKFAVIRHQQSLLYKEYLSEKETWKTESKTIKEEKRKLEDQVQQDAIKVKEYNNLLNALQMDSDEMKKILAENSRKITVLQVNEKSLIRQYTTLVELERQLRKENEKQKNELLSMEAEVCEKIGCLQRFKEMAIFKIAALQKVVDNSVSLSELELANKQYNELTAKYRDILQKDNMLVQRTSNLEHLECENISLKEQVESINKELEITKEKLHTIEQAWEQETKLGNESSMDKAKKSITNSDIVSISKKITMLEMKELNERQRAEHCQKMYEHLRTSLKQMEERNFELETKFAELTKINLDAQKVEQMLRDELADSVSKAVSDADRQRILELEKNEMELKVEVSKLREISDIARRQVEILNAQQQSRDKEV

SEQ ID NO: 4 - protein, 515 aa, Homo sapiens
ESLRMQLLDYQAQSDEKSLIAKLHQHNVSLQLSEATALGKLESITSKLQKMEAYNLRLEQKLDEKEQALYYARLEGRNRAKHLRQTIQSLRRQFSGALPLAQQEKFSKTMIQLQNDKLKIMQEMKNSQQEHRNMENKTLEMELKLKGLEELISTLKDTKGAQKVINWHMKIEELRLQELKLNRELVKDKEEIKYLNNIISEYERTISSLEEEIVQQNKFHEERQMAWDQREVDLERQLDIFDRQQNEILNAAQKFEEATGSIPDPSLPLPNQLEIALRKIKENIRIILETRATCKSLEEKLKEKESALRLAEQNILSRDKVINELRLRLPATAEREKLIAELGRKEMEPKSHHTLKIAHQTIANMQARLNQKEEVLKKYQRLLEKAREEQREIVKKHEEDLHILHHRLELQADSSLNKFKQTAWDLMKQSPTPVPTNKHFIRLAEMEQTVAEQDDSLSSLLVKLKKVSQDLERQREITELKVKEFENIKLQLQENHEDEVKKVKAEVEDLKYLLD

SEQ ID NO: 5 - DNA, 3606 bp, Homo sapiens
actgaaaacatttctcaaggagatagaataagtgaaagaaaattggatttattgagcctcaaaaatatgagtgaagcacaatcaaagaatgaatttctttcaagagaactaattgaaaaagaaagagatttagaaaggagtaggacagtgatagccaaatttcagaataaattaaaagaattagttgaagaaaataagcaacttgaagaaggtatgaaagaaatattgcaagcaattaaggaaatgcagaaagatcctgatgttaaaggaggagaaacatctctaattatccctagccttgaaagactagttaatgctatagaatcaaagaatgcagaaggaatctttgatgcgagtctgcatttgaaagcccaagttgatcagcttaccggaagaaatgaagaattaagacaggagctcagggaatctcggaaagaggctataaattattcacagcagttggcaaaagctaatttaaagatagaccatcttgaaaaagaaactagtcttttacgacaatcagaaggatcgaatgttgtttttaaaggaattgacttacctgatgggatagcaccatctagtgccagtatcattaattctcagaatgaatatttaatacatttgttacaggaactagaaaataaagaaaaaaagttaaagaatttagaagattctcttgaagattacaacagaaaatttgctgtaattcgtcatcaacaaagtttgttgtataaagaatacctaagtgaaaaggagacctggaaaacagaatctaaaacaataaaagaggaaaagagaaaacttgaggatcaagtccaacaagatgctataaaagtaaaagaatataataatttgctcaatgctcttcagatggattcggatgaaatgaaaaaaatacttgcagaaaatagtaggaaaattactgttttgcaagtgaatgaaaaatcacttataaggcaatatacaaccttagtagaattggagcgacaacttagaaaagaaaatgagaagcaaaagaatgaattgttgtcaatggaggctgaagtttgtgaaaaaattgggtgtttgcaaagatttaaggaaatggccattttcaagattgcagctctccaaaaagttgtagataatagtgtttctttgtctgaactagaactggctaataaacagtacaatgaactgactgctaagtacagggacatcttgcaaaaagataatatgcttgttcaaagaacaagtaacttggaacacctggagtgtgaaaacatctccttaaaagaacaagtggagtctataaataaagaactggagattaccaaggaaaaacttcacactattgaacaagcctgggaacaggaaactaaattaggtaatgaatctagcatggataaggcaaagaaatcaataaccaacagtgacattgtttccatttcaaaaaaaataactatgctggaaatgaaggaattaaatgaaaggcagcgggctgaacattgtcaaaaaatgtatgaacacttacggacttcgttaaagcaaatggaggaacgtaattttgaattggaaaccaaatttgctgagcttaccaaaatcaatttggatgcacagaaggtggaacagatgttaagagatgaattagctgatagtgtgagcaaggcagtaagtgatgctgataggcaacggattctagaattagagaagaatgaaatggaactaaaagttgaagtgtcaaaactgagagagatttctgatattgccagaagacaagttgaaattttgaatgcacaacaacaatctagggacaaggaagtaactgaaaacatttctcaaggagatagaataagtgaaagaaaattggatttattgagcctcaaaaatatgagtgaagcacaatcaaagaatgaatttctttcaagagaactaattgaaaaagaaagagatttagaaaggagtaggacagtgatagccaaatttcagaataaattaaaagaattagttgaagaaaataagcaacttgaagaaggtatgaaagaaatattgcaagcaattaaggaaatgcagaaagatcctgatgttaaaggaggagaaacatctctaattatccctagccttgaaagactagttaatgctatagaatcaaagaatgcagaaggaatctttgatgcgagtctgcatttgaaagcccaagttgatcagcttaccggaagaaatgaagaattaagacaggagctcagggaatctcggaaagaggctataaattattcacagcagttggcaaaagctaatttaaagatagaccatcttgaaaaagaaactagtcttttacgacaatcagaaggatcgaatgttgtttttaaaggaattgacttacctgatgggatagcaccatctagtgccagtatcattaattctcagaatgaatatttaatacatttgttacaggaactagaaaataaagaaaaaaagttaaagaatttagaagattctcttgaagattacaacagaaaatttgctgtaattcgtcatcaacaaagtttgttgtataaagaatacctaagtgaaaaggagacctggaaaacagaatctaaaacaataaaagaggaaaagagaaaacttgaggatcaagtccaacaagatgctataaaagtaaaagaatataataatttgctcaatgctcttcagatggattcggatgaaatgaaaaaaatacttgcagaaaatagtaggaaaattactgttttgcaagtgaatgaaaaatcacttataaggcaatatacaaccttagtagaattggagcgacaacttagaaaagaaaatgagaagcaaaagaatgaattgttgtcaatggaggctgaagtttgtgaaaaaattgggtgtttgcaaagatttaaggaaatggccattttcaagattgcagctctccaaaaagttgtagataatagtgtttctttgtctgaactagaactggctaataaacagtacaatgaactgactgctaagtacagggacatcttgcaaaaagataatatgcttgttcaaagaacaagtaacttggaacacctggagtgtgaaaacatctccttaaaagaacaagtggagtctataaataaagaactggagattaccaaggaaaaacttcacactattgaacaagcctgggaacaggaaactaaattaggtaatgaatctagcatggataaggcaaagaaatcaataaccaacagtgacattgtttccatttcaaaaaaaataactatgctggaaatgaaggaattaaatgaaaggcagcgggctgaacattgtcaaaaaatgtatgaacacttacggacttcgttaaagcaaatggaggaacgtaattttgaattggaaaccaaatttgctgagcttaccaaaatcaatttggatgcacagaaggtggaacagatgttaagagatgaattagctgatagtgtgagcaaggcagtaagtgatgctgataggcaacggattctagaattagagaagaatgaaatggaactaaaagttgaagtgtcaaaactgagagagatttctgatattgccagaagacaagttgaaattttgaatgcacaacaacaatctagggacaaggaagta

SEQ ID NO: 6 - DNA, 1803 bp, Homo sapiens
actgaaaacatttctcaaggagatagaataagtgaaagaaaattggatttattgagcctcaaaaatatgagtgaagcacaatcaaagaatgaatttctttcaagagaactaattgaaaaagaaagagatttagaaaggagtaggacagtgatagccaaatttcagaataaattaaaagaattagttgaagaaaataagcaacttgaagaaggtatgaaagaaatattgcaagcaattaaggaaatgcagaaagatcctgatgttaaaggaggagaaacatctctaattatccctagccttgaaagactagttaatgctatagaatcaaagaatgcagaaggaatctttgatgcgagtctgcatttgaaagcccaagttgatcagcttaccggaagaaatgaagaattaagacaggagctcagggaatctcggaaagaggctataaattattcacagcagttggcaaaagctaatttaaagatagaccatcttgaaaaagaaactagtcttttacgacaatcagaaggatcgaatgttgtttttaaaggaattgacttacctgatgggatagcaccatctagtgccagtatcattaattctcagaatgaatatttaatacatttgttacaggaactagaaaataaagaaaaaaagttaaagaatttagaagattctcttgaagattacaacagaaaatttgctgtaattcgtcatcaacaaagtttgttgtataaagaatacctaagtgaaaaggagacctggaaaacagaatctaaaacaataaaagaggaaaagagaaaacttgaggatcaagtccaacaagatgctataaaagtaaaagaatataataatttgctcaatgctcttcagatggattcggatgaaatgaaaaaaatacttgcagaaaatagtaggaaaattactgttttgcaagtgaatgaaaaatcacttataaggcaatatacaaccttagtagaattggagcgacaacttagaaaagaaaatgagaagcaaaagaatgaattgttgtcaatggaggctgaagtttgtgaaaaaattgggtgtttgcaaagatttaaggaaatggccattttcaagattgcagctctccaaaaagttgtagataatagtgtttctttgtctgaactagaactggctaataaacagtacaatgaactgactgctaagtacagggacatcttgcaaaaagataatatgcttgttcaaagaacaagtaacttggaacacctggagtgtgaaaacatctccttaaaagaacaagtggagtctataaataaagaactggagattaccaaggaaaaacttcacactattgaacaagcctgggaacaggaaactaaattaggtaatgaatctagcatggataaggcaaagaaatcaataaccaacagtgacattgtttccatttcaaaaaaaataactatgctggaaatgaaggaattaaatgaaaggcagcgggctgaacattgtcaaaaaatgtatgaacacttacggacttcgttaaagcaaatggaggaacgtaattttgaattggaaaccaaatttgctgagcttaccaaaatcaatttggatgcacagaaggtggaacagatgttaagagatgaattagctgatagtgtgagcaaggcagtaagtgatgctgataggcaacggattctagaattagagaagaatgaaatggaactaaaagttgaagtgtcaaaactgagagagatttctgatattgccagaagacaagttgaaattttgaatgcacaacaacaatctagggacaaggaagta

SEQ ID NO: 7 - DNA, 1545 bp, Homo sapiens
gagtccctcagaatgcaactgctagactatcaggcacagtctgatgaaaagtcgctcattgccaagttgcaccaacataatgtctctcttcaactgagtgaggctactgctcttggtaagttggagtcaattacatctaaactgcagaagatggaggcctacaacttgcgcttagagcagaaacttgatgaaaaagaacaggctctctattatgctcgtttggagggaagaaacagagcaaaacatctgcgccaaacaattcagtctctacgacgacagtttagtggagctttacccttggcacaacaggaaaagttctccaaaacaatgattcaactacaaaatgacaaacttaagataatgcaagaaatgaaaaattctcaacaagaacatagaaatatggagaacaaaacattggagatggaattaaaattaaagggcctggaagagttaataagcactttaaaggataccaaaggagcccaaaaggtaatcaactggcatatgaaaatagaagaacttcgtcttcaagaacttaaactaaatcgggaattagtcaaggataaagaagaaataaaatatttgaataacataatttctgaatatgaacgtacaatcagcagtcttgaagaagaaattgtgcaacagaacaagtttcatgaagaaagacaaatggcctgggatcaaagagaagttgacctggaacgccaactagacatttttgaccgtcagcaaaatgaaatactaaatgcggcacaaaagtttgaagaagctacaggatcaatccctgaccctagtttgccccttccaaatcaacttgagatcgctctaaggaaaattaaggagaacattcgaataattctagaaacacgggcaacttgcaaatcactagaagagaaactaaaagagaaagaatctgctttaaggttagcagaacaaaatatactgtcaagagacaaagtaatcaatgaactgaggcttcgattgcctgccactgcagaaagagaaaagctcatagctgagctaggcagaaaagagatggaaccaaaatctcaccacacattgaaaattgctcatcaaaccattgcaaacatgcaagcaaggttaaatcaaaaagaagaagtattaaagaagtatcaacgtcttctagaaaaagccagagaggagcaaagagaaattgtgaagaaacatgaggaagaccttcatattcttcatcacagattagaactacaggctgatagttcactaaataaattcaaacaaacggcttgggatttaatgaaacagtctcccactccagttcctaccaacaagcattttattcgtctggctgagatggaacagacagtagcagaacaagatgactctctttcctcactcttggtcaaactaaagaaagtatcacaagatttggagagacaaagagaaatcactgaattaaaagtaaaagaatttgaaaatatcaaattacagcttcaagaaaaccatgaagatgaagtgaaaaaagtaaaagcggaagtagaggatttaaagtatcttctggac

SEQ ID NO: 8 - DNA, 7972 bp, Homo sapiens
atttgaagtcctcgttccacgccttctcatcatcctgaacaccgagctctgggactccggcggagaatctaaacgtaaagcatcacccacggtcgtgaactgtaggctctcctggcatccgggatcttattctggccttggcggagttggggatggtgtcgcctagcagccgctgccgctttggcttgctcgggaccatttggctggacccagagtccgcgtggaaccgcgatagggatctgtcagggcccgcggccgggtccagcttggtggttgcggtagtgagaggcctccgctggttgccaggcttggtctagaggtggagcacagtgaaagaattcaagatgccacctaatataaactggaaagaaataatgaaagttgacccagatgacctgccccgtcaagaagaactggcagataatttattgatttccttatccaaggtggaagtaaatgagctaaaaagtgaaaagcaagaaaatgtgatacaccttttcagaattactcagtcactaatgaagatgaaagctcaagaagtggagctggctttggaagaagtagaaaaagctggagaagaacaagcaaaatttgaaaatcaattaaaaactaaagtaatgaaactggaaaatgaactggagatggctcagcagtctgcaggtggacgagatactcggtttttacgtaatgaaatttgccaacttgaaaaacaattagaacaaaaagatagagaattggaggacatggaaaaggagttggagaaagagaagaaagttaatgagcaattggctcttcgaaatgaggaggcagaaaatgaaaacagcaaattaagaagagagaacaaacgtctaaagaaaaagaatgaacaactttgtcaggatattattgactaccagaaacaaatagattcacagaaagaaacacttttatcaagaagaggggaagacagtgactaccgatcacagttgtctaaaaaaaactatgagcttatccaatatcttgatgaaattcagactttaacagaagctaatgagaaaattgaagttcagaatcaagaaatgagaaaaaatttagaagagtctgtacaggaaatggagaagatgactgatgaatataatagaatgaaagctattgtgcatcagacagataatgtaatagatcagttaaaaaaagaaaacgatcattatcaacttcaagtgcaggagcttacagatcttctgaaatcaaaaaatgaagaagatgatccaattatggtagctgtcaatgcaaaagtagaagaatggaagctaattttgtcttctaaagatgatgaaattattgagtatcagcaaatgttacataacctaagggagaaacttaagaatgctcagcttgatgctgataaaagtaatgttatggctctacagcagggtatacaggaacgagacagtcaaattaagatgctcaccgaacaagtagaacaatatacaaaagaaatggaaaagaatacttgtattattgaagatttgaaaaatgagctccaaagaaacaaaggtgcttcaaccctttctcaacagactcatatgaaaattcagtcaacgttagacattttaaaagagaaaactaaagaggctgagagaacagctgaactggctgaggctgatgctagggaaaaggataaagaattagttgaggctctgaagaggttaaaagattatgaatcgggagtatatggtttagaagatgctgtcgttgaaataaagaattgtaaaaaccaaattaaaataagagatcgagagattgaaatattaacaaaggaaatcaataaacttgaattgaagatcagtgatttccttgatgaaaatgaggcacttagagagcgtgtgggccttgaaccaaagacaatgattgatttaactgaatttagaaatagcaaacacttaaaacagcagcagtacagagctgaaaaccagattcttttgaaagagattgaaagtctagaggaagaacgacttgatctgaaaaaaaaaattcgtcaaatggctcaagaaagaggaaaaagaagtgcaacttcaggattaaccactgaggacctgaacctaactgaaaacatttctcaaggagatagaataagtgaaagaaaattggatttattgagcctcaaaaatatgagtgaagcacaatcaaagaatgaatttctttcaagagaactaattgaaaaagaaagagatttagaaaggagtaggacagtgatagccaaatttcagaataaattaaaagaattagttgaagaaaataagcaacttgaagaaggtatgaaagaaatattgcaagcaattaaggaaatgcagaaagatcctgatgttaaaggaggagaaacatctctaattatccctagccttgaaagactagttaatgctatagaatcaaagaatgcagaaggaatctttgatgcgagtctgcatttgaaagcccaagttgatcagcttaccggaagaaatgaagaattaagacaggagctcagggaatctcggaaagaggctataaattattcacagcagttggcaaaagctaatttaaagatagaccatcttgaaaaagaaactagtcttttacgacaatcagaaggatcgaatgttgtttttaaaggaattgacttacctgatgggatagcaccatctagtgccagtatcattaattctcagaatgaatatttaatacatttgttacaggaactagaaaataaagaaaaaaagttaaagaatttagaagattctcttgaagattacaacagaaaatttgctgtaattcgtcatcaacaaagtttgttgtataaagaatacctaagtgaaaaggagacctggaaaacagaatctaaaacaataaaagaggaaaagagaaaacttgaggatcaagtccaacaagatgctataaaagtaaaagaatataataatttgctcaatgctcttcagatggattcggatgaaatgaaaaaaatacttgcagaaaatagtaggaaaattactgttttgcaagtgaatgaaaaatcacttataaggcaatatacaaccttagtagaattggagcgacaacttagaaaagaaaatgagaagcaaaagaatgaattgttgtcaatggaggctgaagtttgtgaaaaaattgggtgtttgcaaagatttaaggaaatggccattttcaagattgcagctctccaaaaagttgtagataatagtgtttctttgtctgaactagaactggctaataaacagtacaatgaactgactgctaagtacagggacatcttgcaaaaagataatatgcttgttcaaagaacaagtaacttggaacacctggagtgtgaaaacatctccttaaaagaacaagtggagtctataaataaagaactggagattaccaaggaaaaacttcacactattgaacaagcctgggaacaggaaactaaattaggtaatgaatctagcatggataaggcaaagaaatcaataaccaacagtgacattgtttccatttcaaaaaaaataactatgctggaaatgaaggaattaaatgaaaggcagcgggctgaacattgtcaaaaaatgtatgaacacttacggacttcgttaaagcaaatggaggaacgtaattttgaattggaaaccaaatttgctgagcttaccaaaatcaatttggatgcacagaaggtggaacagatgttaagagatgaattagctgatagtgtgagcaaggcagtaagtgatgctgataggcaacggattctagaattagagaagaatgaaatggaactaaaagttgaagtgtcaaaactgagagagatttctgatattgccagaagacaagttgaaattttgaatgcacaacaacaatctagggacaaggaagtagagtccctcagaatgcaactgctagactatcaggcacagtctgatgaaaagtcgctcattgccaagttgcaccaacataatgtctctcttcaactgagtgaggctactgctcttggtaagttggagtcaattacatctaaactgcagaagatggaggcctacaacttgcgcttagagcagaaacttgatgaaaaagaacaggctctctattatgctcgtttggagggaagaaacagagcaaaacatctgcgccaaacaattcagtctctacgacgacagtttagtggagctttacccttggcacaacaggaaaagttctccaaaacaatgattcaactacaaaatgacaaacttaagataatgcaagaaatgaaaaattctcaacaagaacatagaaatatggagaacaaaacattggagatggaattaaaattaaagggcctggaagagttaataagcactttaaaggataccaaaggagcccaaaaggtaatcaactggcatatgaaaatagaagaacttcgtcttcaagaacttaaactaaatcgggaattagtcaaggataaagaagaaataaaatatttgaataacataatttctgaatatgaacgtacaatcagcagtcttgaagaagaaattgtgcaacagaacaagtttcatgaagaaagacaaatggcctgggatcaaagagaagttgacctggaacgccaactagacatttttgaccgtcagcaaaatgaaatactaaatgcggcacaaaagtttgaagaagctacaggatcaatccctgaccctagtttgccccttccaaatcaacttgagatcgctctaaggaaaattaaggagaacattcgaataattctagaaacacgggcaacttgcaaatcactagaagagaaactaaaagagaaagaatctgctttaaggttagcagaacaaaatatactgtcaagagacaaagtaatcaatgaactgaggcttcgattgcctgccactgcagaaagagaaaagctcatagctgagctaggcagaaaagagatggaaccaaaatctcaccacacattgaaaattgctcatcaaaccattgcaaacatgcaagcaaggttaaatcaaaaagaagaagtattaaagaagtatcaacgtcttctagaaaaagccagagaggagcaaagagaaattgtgaagaaacatgaggaagaccttcatattcttcatcacagattagaactacaggctgatagttcactaaataaattcaaacaaacggcttgggatttaatgaaacagtctcccactccagttcctaccaacaagcattttattcgtctggctgagatggaacagacagtagcagaacaagatgactctctttcctcactcttggtcaaactaaagaaagtatcacaagatttggagagacaaagagaaatcactgaattaaaagtaaaagaatttgaaaatatcaaattacagcttcaagaaaaccatgaagatgaagtgaaaaaagtaaaagcggaagtagaggatttaaagtatcttctggaccagtcacaaaaggagtcacagtgtttaaaatctgaacttcaggctcaaaaagaagcaaattcaagagctccaacaactacaatgagaaatctagtagaacggctaaagagccaattagccttgaaggagaaacaacagaaagcacttagtcgggcacttttagaactccgggcagaaatgacagcagctgctgaagaacgtattatttctgcaacttctcaaaaagaggcccatctcaatgttcaacaaatcgttgatcgacatactagagagctaaagacacaagttgaagatttaaatgaaaatcttttaaaattgaaagaagcacttaaaacaagtaaaaacagagaaaactcactaactgataatttgaatgacttaaataatgaactgcaaaagaaacaaaaagcctataataaaatacttagagagaaagaggaaattgatcaagagaatgatgaactgaaaaggcaaattaaaagactaaccagtggattacagggcaaacccctgacagataataaacaaagtctaattgaagaactccaaaggaaagttaaaaaactagagaaccaattagagggaaaggtggaggaagtagacctaaaacctatgaaagaaaagaatgctaaagaagaattaattaggtgggaagaaggtaaaaagtggcaagccaaaatagaaggaattcgaaacaagttaaaagagaaagagggggaagtctttactttaacaaagcagttgaatactttgaaggatctttttgccaaagccgataaagagaaacttactttgcagaggaaactaaaaacaactggcatgactgttgatcaggttttgggaatacgagctttggagtcagaaaaagaattggaagaattaaaaaagagaaatcttgacttagaaaatgatatattgtatatgagggcccaccaagctcttcctcgagattctgttgtagaagatttacatttacaaaatagatacctccaagaaaaacttcatgctttagaaaaacagttttcaaaggatacatattctaagccttcaatttcaggaatagagtcagatgatcattgtcagagagaacaggagcttcagaaggaaaacttgaagttgtcatctgaaaatattgaactgaaatttcagcttgaacaagcaaataaagatttgccaagattaaagaatcaagtcagagatttgaaggaaatgtgtgaatttcttaagaaagaaaaagcagaagttcagcggaaacttggccatgttagagggtctggtagaagtggaaagacaatcccagaactggaaaaaaccattggtttaatgaaaaaagtagttgaaaaagtccagagagaaaatgaacagttgaaaaaagcatcaggaatattgactagtgaaaaaatggctaatattgagcaggaaaatgaaaaattgaaggctgaattagaaaaacttaaagctcatcttgggcatcagttgagcatgcactatgaatccaagaccaaaggcacagaaaaaattattgctgaaaatgaaaggcttcgtaaagaacttaaaaaagaaactgatgctgcagagaaattacggatagcaaagaataatttagagatattaaatgagaagatgacagttcaactagaagagactggtaagagattgcagtttgcagaaagcagaggtccacagcttgaaggtgctgacagtaagagctggaaatccattgtggttacaagaatgtatgaaaccaagttaaaagaattggaaactgatattgccaaaaaaaatcaaagcattactgaccttaaacagcttgtaaaagaagcaacagagagagaacaaaaagttaacaaatacaatgaagaccttgaacaacagattaagattcttaaacatgttcctgaaggtgctgagacagagcaaggccttaaacgggagcttcaagttcttagattagctaatcatcagctggataaagagaaagcagaattaatccatcagatagaagctaacaaggaccaaagtggagctgaaagcaccatacctgatgctgatcaactaaaggaaaaaataaaagatctagagacacagctcaaaatgtcagatctagaaaagcagcatttgaaggaggaaataaagaagctgaaaaaagaactggaaaattttgatccttcattttttgaagaaattgaagatcttaagtataattacaaggaagaagtgaagaagaatattctcttagaagagaaggtaaaaaaactttcagaacaattgggagttgaattaactagccctgttgctgcttctgaagagtttgaagatgaagaagaaagtcctgttaatttccccatttactaaaggtcacctataaactttgtttcatttaactatttattaactttataagttaaatatacttggaaataagcagttctccgaactgtagtatttccttctcactaccttgtacctttatacttagattggaattcttaataaataaaattatatgaaattttcaacttattaaaaaaaaaaaaaaaaaa

SEQ ID NO: 9 - protein, 738 aa, Unknown
  AAV8 capsid protein
MAADGYLPDWLEDNLSEGIREWWALKPGAPKPKANQQKQDDGRGLVLPGYKYLGPFNGLDKGEPVNAADAAALEHDKAYDQQLQAGDNPYLRYNHADAEFQERLQEDTSFGGNLGRAVFQAKKRVLEPLGLVEEGAKTAPGKKRPVEPSPQRSPDSSTGIGKKGQQPARKRLNFGQTGDSESVPDPQPLGEPPAAPSGVGPNTMAAGGGAPMADNNEGADGVGSSSGNWHCDSTWLGDRVITTSTRTWALPTYNNHLYKQISNGTSGGATNDNTYFGYSTPWGYFDFNRFHCHFSPRDWQRLINNNWGFRPKRLSFKLFNIQVKEVTQNEGTKTIANNLTSTIQVFTDSEYQLPYVLGSAHQGCLPPFPADVFMIPQYGYLTLNNGSQAVGRSSFYCLEYFPSQMLRTGNNFQFTYTFEDVPFHSSYAHSQSLDRLMNPLIDQYLYYLSRTQTTGGTANTQTLGFSQGGPNTMANQAKNWLPGPCYRQQRVSTTTGQNNNSNFAWTAGTKYHLNGRNSLANPGIAMATHKDDEERFFPSNGILIFGKQNAARDNADYSDVMLTSEEEIKTTNPVATEEYGIVADNLQQQNTAPQIGTVNSQGALPGMVWQNRDVYLQGPIWAKIPHTDGNFHPSPLMGGFGLKHPPPQILIKNTPVPADPPTTFNQSKLNSFITQYSTGQVSVEIEWELQKENSKRWNPEIQYTSNYYKSTSVDFAVNTEGVYSEPRPIGTRYLTRNL

SEQ ID NO: 10 - protein, 1299 aa, Homo sapiens
ESLRMQLLDYQAQSDEKSLIAKLHQHNVSLQLSEATALGKLESITSKLQKMEAYNLRLEQKLDEKEQALYYARLEGRNRAKHLRQTIQSLRRQFSGALPLAQQEKFSKTMIQLQNDKLKIMQEMKNSQQEHRNMENKTLEMELKLKGLEELISTLKDTKGAQKVINWHMKIEELRLQELKLNRELVKDKEEIKYLNNIISEYERTISSLEEEIVQQNKFHEERQMAWDQREVDLERQLDIFDRQQNEILNAAQKFEEATGSIPDPSLPLPNQLEIALRKIKENIRIILETRATCKSLEEKLKEKESALRLAEQNILSRDKVINELRLRLPATAEREKLIAELGRKEMEPKSHHTLKIAHQTIANMQARLNQKEEVLKKYQRLLEKAREEQREIVKKHEEDLHILHHRLELQADSSLNKFKQTAWDLMKQSPTPVPTNKHFIRLAEMEQTVAEQDDSLSSLLVKLKKVSQDLERQREITELKVKEFENIKLQLQENHEDEVKKVKAEVEDLKYLLDQSQKESQCLKSELQAQKEANSRAPTTTMRNLVERLKSQLALKEKQQKALSRALLELRAEMTAAAEERIISATSQKEAHLNVQQIVDRHTRELKTQVEDLNENLLKLKEALKTSKNRENSLTDNLNDLNNELQKKQKAYNKILREKEEIDQENDELKRQIKRLTSGLQGKPLTDNKQSLIEELQRKVKKLENQLEGKVEEVDLKPMKEKNAKEELIRWEEGKKWQAKIEGIRNKLKEKEGEVFTLTKQLNTLKDLFAKADKEKLTLQRKLKTTGMTVDQVLGIRALESEKELEELKKRNLDLENDILYMRAHQALPRDSVVEDLHLQNRYLQEKLHALEKQFSKDTYSKPSISGIESDDHCQREQELQKENLKLSSENIELKFQLEQANKDLPRLKNQVRDLKEMCEFLKKEKAEVQRKLGHVRGSGRSGKTIPELEKTIGLMKKVVEKVQRENEQLKKASGILTSEKMANIEQENEKLKAELEKLKAHLGHQLSMHYESKTKGTEKIIAENERLRKELKKETDAAEKLRIAKNNLEILNEKMTVQLEETGKRLQFAESRGPQLEGADSKSWKSIVVTRMYETKLKELETDIAKKNQSITDLKQLVKEATEREQKVNKYNEDLEQQIKILKHVPEGAETEQGLKRELQVLRLANHQLDKEKAELIHQIEANKDQSGAESTIPDADQLKEKIKDLETQLKMSDLEKQHLKEEIKKLKKELENFDPSFFEEIEDLKYNYKEEVKKNILLEEKVKKLSEQLGVELTSPVAASEEFEDEEESPVNFPIY

SEQ ID NO: 11 - protein, 400 aa, Homo sapiens
ILTKEINKLELKISDFLDENEALRERVGLEPKTMIDLTEFRNSKHLKQQQYRAENQILLKEIESLEEERLDLKKKIRQMAQERGKRSATSGLTTEDLNLTENISQGDRISERKLDLLSLKNMSEAQSKNEFLSRELIEKERDLERSRTVIAKFQNKLKELVEENKQLEEGMKEILQAIKEMQKDPDVKGGETSLIIPSLERLVNAIESKNAEGIFDASLHLKAQVDQLTGRNEELRQELRESRKEAINYSQQLAKANLKIDHLEKETSLLRQSEGSNVVFKGIDLPDGIAPSSASIINSQNEYLIHLLQELENKEKKLKNLEDSLEDYNRKFAVIRHQQSLLYKEYLSEKETWKTESKTIKEEKRKLEDQVQQDAIKVKEYNNLLNALQMDSDEMKKILA

SEQ ID NO: 12 - protein, 1029 aa, Homo sapiens
ESLRMQLLDYQAQSDEKSLIAKLHQHNVSLQLSEATALGKLESITSKLQKMEAYNLRLEQKLDEKEQALYYARLEGRNRAKHLRQTIQSLRRQFSGALPLAQQEKFSKTMIQLQNDKLKIMQEMKNSQQEHRNMENKTLEMELKLKGLEELISTLKDTKGAQKVINWHMKIEELRLQELKLNRELVKDKEEIKYLNNIISEYERTISSLEEEIVQQNKFHEERQMAWDQREVDLERQLDIFDRQQNEILNAAQKFEEATGSIPDPSLPLPNQLEIALRKIKENIRIILETRATCKSLEEKLKEKESALRLAEQNILSRDKVINELRLRLPATAEREKLIAELGRKEMEPKSHHTLKIAHQTIANMQARLNQKEEVLKKYQRLLEKAREEQREIVKKHEEDLHILHHRLELQADSSLNKFKQTAWDLMKQSPTPVPTNKHFIRLAEMEQTVAEQDDSLSSLLVKLKKVSQDLERQREITELKVKEFENIKLQLQENHEDEVKKVKAEVEDLKYLLDTTGMTVDQVLGIRALESEKELEELKKRNLDLENDILYMRAHQALPRDSVVEDLHLQNRYLQEKLHALEKQFSKDTYSKPSISGIESDDHCQREQELQKENLKLSSENIELKFQLEQANKDLPRLKNQVRDLKEMCEFLKKEKAEVQRKLGHVRGSGRSGKTIPELEKTIGLMKKVVEKVQRENEQLKKASGILTSEKMANIEQENEKLKAELEKLKAHLGHQLSMHYESKTKGTEKIIAENERLRKELKKETDAAEKLRIAKNNLEILNEKMTVQLEETGKRLQFAESRGPQLEGADSKSWKSIVVTRMYETKLKELETDIAKKNQSITDLKQLVKEATEREQKVNKYNEDLEQQIKILKHVPEGAETEQGLKRELQVLRLANHQLDKEKAELIHQIEANKDQSGAESTIPDADQLKEKIKDLETQLKMSDLEKQHLKEEIKKLKKELENFDPSFFEEIEDLKYNYKEEVKKNILLEEKVKKLSEQLGVELTSPVAASEEFEDEEESPVNFPIY

SEQ ID NO: 13 - protein, 1281 aa, Homo sapiens
TENISQGDRISERKLDLLSLKNMSEAQSKNEFLSRELIEKERDLERSRTVIAKFQNKLKELVEENKQLEEGMKEILQAIKEMQKDPDVKGGETSLIIPSLERLVNAIESKNAEGIFDASLHLKAQVDQLTGRNEELRQELRESRKEAINYSQQLAKANLKIDHLEKETSLLRQSEGSNVVFKGIDLPDGIAPSSASIINSQNEYLIHLLQELENKEKKLKNLEDSLEDYNRKFAVIRHQQSLLYKEYLSEKETWKTESKTIKEEKRKLEDQVQQDAIKVKEYNNLLNALQMDSDEMKKILAENSRKITVLQVNEKSLIRQYTTLVELERQLRKENEKQKNELLSMEAEVCEKIGCLQRFKEMAIFKIAALQKVVDNSVSLSELELANKQYNELTAKYRDILQKDNMLVQRTSNLEHLECENISLKEQVESINKELEITKEKLHTIEQAWEQETKLGNESSMDKAKKSITNSDIVSISKKITMLEMKELNERQRAEHCQKMYEHLRTSLKQMEERNFELETKFAELTKINLDAQKVEQMLRDELADSVSKAVSDADRQRILELEKNEMELKVEVSKLREISDIARRQVEILNAQQQSRDKEVKLKEALKTSKNRENSLTDNLNDLNNELQKKQKAYNKILREKEEIDQENDELKRQIKRLTSGLQGKPLTDNKQSLIEELQRKVKKLENQLEGKVEEVDLKPMKEKNAKEELIRWEEGKKWQAKIEGIRNKLKEKEGEVFTLTKQLNTLKDLFAKADKEKLTLQRKLKTTGMTVDQVLGIRALESEKELEELKKRNLDLENDILYMRAHQALPRDSVVEDLHLQNRYLQEKLHALEKQFSKDTYSKPSISGIESDDHCQREQELQKENLKLSSENIELKFQLEQANKDLPRLKNQVRDLKEMCEFLKKEKAEVQRKLGHVRGSGRSGKTIPELEKTIGLMKKVVEKVQRENEQLKKASGILTSEKMANIEQENEKLKAELEKLKAHLGHQLSMHYESKTKGTEKIIAENERLRKELKKETDAAEKLRIAKNNLEILNEKMTVQLEETGKRLQFAESRGPQLEGADSKSWKSIVVTRMYETKLKELETDIAKKNQSITDLKQLVKEATEREQKVNKYNEDLEQQIKILKHVPEGAETEQGLKRELQVLRLANHQLDKEKAELIHQIEANKDQSGAESTIPDADQLKEKIKDLETQLKMSDLEKQHLKEEIKKLKKELENFDPSFFEEIEDLKYNYKEEVKKNILLEEKVKKLSEQLGVELTSPVAASEEFEDEEESPVNFPIY

SEQ ID NO: 14 - protein, 786 aa, Homo sapiens
ESLRMQLLDYQAQSDEKSLIAKLHQHNVSLQLSEATALGKLESITSKLQKMEAYNLRLEQKLDEKEQALYYARLEGRNRAKHLRQTIQSLRRQFSGALPLAQQEKFSKTMIQLQNDKLKIMQEMKNSQQEHRNMENKTLEMELKLKGLEELISTLKDTKGAQKVINWHMKIEELRLQELKLNRELVKDKEEIKYLNNIISEYERTISSLEEEIVQQNKFHEERQMAWDQREVDLERQLDIFDRQQNEILNAAQKFEEATGSIPDPSLPLPNQLEIALRKIKENIRIILETRATCKSLEEKLKEKESALRLAEQNILSRDKVINELRLRLPATAEREKLIAELGRKEMEPKSHHTLKIAHQTIANMQARLNQKEEVLKKYQRLLEKAREEQREIVKKHEEDLHILHHRLELQADSSLNKFKQTAWDLMKQSPTPVPTNKHFIRLAEMEQTVAEQDDSLSSLLVKLKKVSQDLERQREITELKVKEFENIKLQLQENHEDEVKKVKAEVEDLKYLLDQSQKESQCLKSELQAQKEANSRAPTTTMRNLVERLKSQLALKEKQQKALSRALLELRAEMTAAAEERIISATSQKEAHLNVQQIVDRHTRELKTQVEDLNENLLKLKEALKTSKNRENSLTDNLNDLNNELQKKQKAYNKILREKEEIDQENDELKRQIKRLTSGLQGKPLTDNKQSLIEELQRKVKKLENQLEGKVEEVDLKPMKEKNAKEELIRWEEGKKWQAKIEGIRNKLKEKEGEVFTLTKQLNTLKDLFAKADKEKLTLQRKLKT

SEQ ID NO: 15 - protein, 914 aa, Homo sapiens
ILTKEINKLELKISDFLDENEALRERVGLEPKTMIDLTEFRNSKHLKQQQYRAENQILLKEIESLEEERLDLKKKIRQMAQERGKRSATSGLTTEDLNLTENISQGDRISERKLDLLSLKNMSEAQSKNEFLSRELIEKERDLERSRTVIAKFQNKLKELVEENKQLEEGMKEILQAIKEMQKDPDVKGGETSLIIPSLERLVNAIESKNAEGIFDASLHLKAQVDQLTGRNEELRQELRESRKEAINYSQQLAKANLKIDHLEKETSLLRQSEGSNVVFKGIDLPDGIAPSSASIINSQNEYLIHLLQELENKEKKLKNLEDSLEDYNRKFAVIRHQQSLLYKEYLSEKETWKTESKTIKEEKRKLEDQVQQDAIKVKEYNNLLNALQMDSDEMKKILATTGMTVDQVLGIRALESEKELEELKKRNLDLENDILYMRAHQALPRDSVVEDLHLQNRYLQEKLHALEKQFSKDTYSKPSISGIESDDHCQREQELQKENLKLSSENIELKFQLEQANKDLPRLKNQVRDLKEMCEFLKKEKAEVQRKLGHVRGSGRSGKTIPELEKTIGLMKKVVEKVQRENEQLKKASGILTSEKMANIEQENEKLKAELEKLKAHLGHQLSMHYESKTKGTEKIIAENERLRKELKKETDAAEKLRIAKNNLEILNEKMTVQLEETGKRLQFAESRGPQLEGADSKSWKSIVVTRMYETKLKELETDIAKKNQSITDLKQLVKEATEREQKVNKYNEDLEQQIKILKHVPEGAETEQGLKRELQVLRLANHQLDKEKAELIHQIEANKDQSGAESTIPDADQLKEKIKDLETQLKMSDLEKQHLKEEIKKLKKELENFDPSFFEEIEDLKYNYKEEVKKNILLEEKVKKLSEQLGVELTSPVAASEEFEDEEESPVNFPIY

SEQ ID NO: 16 - protein, 885 aa, Homo sapiens
ILTKEINKLELKISDFLDENEALRERVGLEPKTMIDLTEFRNSKHLKQQQYRAENQILLKEIESLEEERLDLKKKIRQMAQERGKRSATSGLTTEDLNLESLRMQLLDYQAQSDEKSLIAKLHQHNVSLQLSEATALGKLESITSKLQKMEAYNLRLEQKLDEKEQALYYARLEGRNRAKHLRQTIQSLRRQFSGALPLAQQEKFSKTMIQLQNDKLKIMQEMKNSQQEHRNMENKTLEMELKLKGLEELISTLKDTKGAQKVINWHMKIEELRLQELKLNRELVKDKEEIKYLNNIISEYERTISSLEEEIVQQNKFHEERQMAWDQREVDLERQLDIFDRQQNEILNAAQKFEEATGSIPDPSLPLPNQLEIALRKIKENIRIILETRATCKSLEEKLKEKESALRLAEQNILSRDKVINELRLRLPATAEREKLIAELGRKEMEPKSHHTLKIAHQTIANMQARLNQKEEVLKKYQRLLEKAREEQREIVKKHEEDLHILHHRLELQADSSLNKFKQTAWDLMKQSPTPVPTNKHFIRLAEMEQTVAEQDDSLSSLLVKLKKVSQDLERQREITELKVKEFENIKLQLQENHEDEVKKVKAEVEDLKYLLDQSQKESQCLKSELQAQKEANSRAPTTTMRNLVERLKSQLALKEKQQKALSRALLELRAEMTAAAEERIISATSQKEAHLNVQQIVDRHTRELKTQVEDLNENLLKLKEALKTSKNRENSLTDNLNDLNNELQKKQKAYNKILREKEEIDQENDELKRQIKRLTSGLQGKPLTDNKQSLIEELQRKVKKLENQLEGKVEEVDLKPMKEKNAKEELIRWEEGKKWQAKIEGIRNKLKEKEGEVFTLTKQLNTLKDLFAKADKEKLTLQRKLKT

SEQ ID NO: 17 - protein, 671 aa, Homo sapiens
ILTKEINKLELKISDFLDENEALRERVGLEPKTMIDLTEFRNSKHLKQQQYRAENQILLKEIESLEEERLDLKKKIRQMAQERGKRSATSGLTTEDLNLTENISQGDRISERKLDLLSLKNMSEAQSKNEFLSRELIEKERDLERSRTVIAKFQNKLKELVEENKQLEEGMKEILQAIKEMQKDPDVKGGETSLIIPSLERLVNAIESKNAEGIFDASLHLKAQVDQLTGRNEELRQELRESRKEAINYSQQLAKANLKIDHLEKETSLLRQSEGSNVVFKGIDLPDGIAPSSASIINSQNEYLIHLLQELENKEKKLKNLEDSLEDYNRKFAVIRHQQSLLYKEYLSEKETWKTESKTIKEEKRKLEDQVQQDAIKVKEYNNLLNALQMDSDEMKKILAQSQKESQCLKSELQAQKEANSRAPTTTMRNLVERLKSQLALKEKQQKALSRALLELRAEMTAAAEERIISATSQKEAHLNVQQIVDRHTRELKTQVEDLNENLLKLKEALKTSKNRENSLTDNLNDLNNELQKKQKAYNKILREKEEIDQENDELKRQIKRLTSGLQGKPLTDNKQSLIEELQRKVKKLENQLEGKVEEVDLKPMKEKNAKEELIRWEEGKKWQAKIEGIRNKLKEKEGEVFTLTKQLNTLKDLFAKADKEKLTLQRKLKT

SEQ ID NO: 18 - protein, 572 aa, Homo sapiens
TENISQGDRISERKLDLLSLKNMSEAQSKNEFLSRELIEKERDLERSRTVIAKFQNKLKELVEENKQLEEGMKEILQAIKEMQKDPDVKGGETSLIIPSLERLVNAIESKNAEGIFDASLHLKAQVDQLTGRNEELRQELRESRKEAINYSQQLAKANLKIDHLEKETSLLRQSEGSNVVFKGIDLPDGIAPSSASIINSQNEYLIHLLQELENKEKKLKNLEDSLEDYNRKFAVIRHQQSLLYKEYLSEKETWKTESKTIKEEKRKLEDQVQQDAIKVKEYNNLLNALQMDSDEMKKILAQSQKESQCLKSELQAQKEANSRAPTTTMRNLVERLKSQLALKEKQQKALSRALLELRAEMTAAAEERIISATSQKEAHLNVQQIVDRHTRELKTQVEDLNENLLKLKEALKTSKNRENSLTDNLNDLNNELQKKQKAYNKILREKEEIDQENDELKRQIKRLTSGLQGKPLTDNKQSLIEELQRKVKKLENQLEGKVEEVDLKPMKEKNAKEELIRWEEGKKWQAKIEGIRNKLKEKEGEVFTLTKQLNTLKDLFAKADKEKLTLQRKLKT

SEQ ID NO: 19 - protein, 801 aa, Homo sapiens
MPPNINWKEIMKVDPDDLPRQEELADNLLISLSKVEVNELKSEKQENVIHLFRITQSLMKMKAQEVELALEEVEKAGEEQAKFENQLKTKVMKLENELEMAQQSAGGRDTRFLRNEICQLEKQLEQKDRELEDMEKELEKEKKVNEQLALRNEEAENENSKLRRENKRLKKKNEQLCQDIIDYQKQIDSQKETLLSRRGETENISQGDRISERKLDLLSLKNMSEAQSKNEFLSRELIEKERDLERSRTVIAKFQNKLKELVEENKQLEEGMKEILQAIKEMQKDPDVKGGETSLIIPSLERLVNAIESKNAEGIFDASLHLKAQVDQLTGRNEELRQELRESRKEAINYSQQLAKANLKIDHLEKETSLLRQSEGSNVVFKGIDLPDGIAPSSASIINSQNEYLIHLLQELENKEKKLKNLEDSLEDYNRKFAVIRHQQSLLYKEYLSEKETWKTESKTIKEEKRKLEDQVQQDAIKVKEYNNLLNALQMDSDEMKKILAENSRKITVLQVNEKSLIRQYTTLVELERQLRKENEKQKNELLSMEAEVCEKIGCLQRFKEMAIFKIAALQKVVDNSVSLSELELANKQYNELTAKYRDILQKDNMLVQRTSNLEHLECENISLKEQVESINKELEITKEKLHTIEQAWEQETKLGNESSMDKAKKSITNSDIVSISKKITMLEMKELNERQRAEHCQKMYEHLRTSLKQMEERNFELETKFAELTKINLDAQKVEQMLRDELADSVSKAVSDADRQRILELEKNEMELKVEVSKLREISDIARRQVEILNAQQQSRDKEV

SEQ ID NO: 20 - DNA, 3900 bp, Homo sapiens
gagtccctcagaatgcaactgctagactatcaggcacagtctgatgaaaagtcgctcattgccaagttgcaccaacataatgtctctcttcaactgagtgaggctactgctcttggtaagttggagtcaattacatctaaactgcagaagatggaggcctacaacttgcgcttagagcagaaacttgatgaaaaagaacaggctctctattatgctcgtttggagggaagaaacagagcaaaacatctgcgccaaacaattcagtctctacgacgacagtttagtggagctttacccttggcacaacaggaaaagttctccaaaacaatgattcaactacaaaatgacaaacttaagataatgcaagaaatgaaaaattctcaacaagaacatagaaatatggagaacaaaacattggagatggaattaaaattaaagggcctggaagagttaataagcactttaaaggataccaaaggagcccaaaaggtaatcaactggcatatgaaaatagaagaacttcgtcttcaagaacttaaactaaatcgggaattagtcaaggataaagaagaaataaaatatttgaataacataatttctgaatatgaacgtacaatcagcagtcttgaagaagaaattgtgcaacagaacaagtttcatgaagaaagacaaatggcctgggatcaaagagaagttgacctggaacgccaactagacatttttgaccgtcagcaaaatgaaatactaaatgcggcacaaaagtttgaagaagctacaggatcaatccctgaccctagtttgccccttccaaatcaacttgagatcgctctaaggaaaattaaggagaacattcgaataattctagaaacacgggcaacttgcaaatcactagaagagaaactaaaagagaaagaatctgctttaaggttagcagaacaaaatatactgtcaagagacaaagtaatcaatgaactgaggcttcgattgcctgccactgcagaaagagaaaagctcatagctgagctaggcagaaaagagatggaaccaaaatctcaccacacattgaaaattgctcatcaaaccattgcaaacatgcaagcaaggttaaatcaaaaagaagaagtattaaagaagtatcaacgtcttctagaaaaagccagagaggagcaaagagaaattgtgaagaaacatgaggaagaccttcatattcttcatcacagattagaactacaggctgatagttcactaaataaattcaaacaaacggcttgggatttaatgaaacagtctcccactccagttcctaccaacaagcattttattcgtctggctgagatggaacagacagtagcagaacaagatgactctctttcctcactcttggtcaaactaaagaaagtatcacaagatttggagagacaaagagaaatcactgaattaaaagtaaaagaatttgaaaatatcaaattacagcttcaagaaaaccatgaagatgaagtgaaaaaagtaaaagcggaagtagaggatttaaagtatcttctggaccagtcacaaaaggagtcacagtgtttaaaatctgaacttcaggctcaaaaagaagcaaattcaagagctccaacaactacaatgagaaatctagtagaacggctaaagagccaattagccttgaaggagaaacaacagaaagcacttagtcgggcacttttagaactccgggcagaaatgacagcagctgctgaagaacgtattatttctgcaacttctcaaaaagaggcccatctcaatgttcaacaaatcgttgatcgacatactagagagctaaagacacaagttgaagatttaaatgaaaatcttttaaaattgaaagaagcacttaaaacaagtaaaaacagagaaaactcactaactgataatttgaatgacttaaataatgaactgcaaaagaaacaaaaagcctataataaaatacttagagagaaagaggaaattgatcaagagaatgatgaactgaaaaggcaaattaaaagactaaccagtggattacagggcaaacccctgacagataataaacaaagtctaattgaagaactccaaaggaaagttaaaaaactagagaaccaattagagggaaaggtggaggaagtagacctaaaacctatgaaagaaaagaatgctaaagaagaattaattaggtgggaagaaggtaaaaagtggcaagccaaaatagaaggaattcgaaacaagttaaaagagaaagagggggaagtctttactttaacaaagcagttgaatactttgaaggatctttttgccaaagccgataaagagaaacttactttgcagaggaaactaaaaacaactggcatgactgttgatcaggttttgggaatacgagctttggagtcagaaaaagaattggaagaattaaaaaagagaaatcttgacttagaaaatgatatattgtatatgagggcccaccaagctcttcctcgagattctgttgtagaagatttacatttacaaaatagatacctccaagaaaaacttcatgctttagaaaaacagttttcaaaggatacatattctaagccttcaatttcaggaatagagtcagatgatcattgtcagagagaacaggagcttcagaaggaaaacttgaagttgtcatctgaaaatattgaactgaaatttcagcttgaacaagcaaataaagatttgccaagattaaagaatcaagtcagagatttgaaggaaatgtgtgaatttcttaagaaagaaaaagcagaagttcagcggaaacttggccatgttagagggtctggtagaagtggaaagacaatcccagaactggaaaaaaccattggtttaatgaaaaaagtagttgaaaaagtccagagagaaaatgaacagttgaaaaaagcatcaggaatattgactagtgaaaaaatggctaatattgagcaggaaaatgaaaaattgaaggctgaattagaaaaacttaaagctcatcttgggcatcagttgagcatgcactatgaatccaagaccaaaggcacagaaaaaattattgctgaaaatgaaaggcttcgtaaagaacttaaaaaagaaactgatgctgcagagaaattacggatagcaaagaataatttagagatattaaatgagaagatgacagttcaactagaagagactggtaagagattgcagtttgcagaaagcagaggtccacagcttgaaggtgctgacagtaagagctggaaatccattgtggttacaagaatgtatgaaaccaagttaaaagaattggaaactgatattgccaaaaaaaatcaaagcattactgaccttaaacagcttgtaaaagaagcaacagagagagaacaaaaagttaacaaatacaatgaagaccttgaacaacagattaagattcttaaacatgttcctgaaggtgctgagacagagcaaggccttaaacgggagcttcaagttcttagattagctaatcatcagctggataaagagaaagcagaattaatccatcagatagaagctaacaaggaccaaagtggagctgaaagcaccatacctgatgctgatcaactaaaggaaaaaataaaagatctagagacacagctcaaaatgtcagatctagaaaagcagcatttgaaggaggaaataaagaagctgaaaaaagaactggaaaattttgatccttcattttttgaagaaattgaagatcttaagtataattacaaggaagaagtgaagaagaatattctcttagaagagaaggtaaaaaaactttcagaacaattgggagttgaattaactagccctgttgctgcttctgaagagtttgaagatgaagaagaaagtcctgttaatttccccatttactaa

SEQ ID NO: 21 - DNA, 1200 bp, Homo sapiens
atattaacaaaggaaatcaataaacttgaattgaagatcagtgatttccttgatgaaaatgaggcacttagagagcgtgtgggccttgaaccaaagacaatgattgatttaactgaatttagaaatagcaaacacttaaaacagcagcagtacagagctgaaaaccagattcttttgaaagagattgaaagtctagaggaagaacgacttgatctgaaaaaaaaaattcgtcaaatggctcaagaaagaggaaaaagaagtgcaacttcaggattaaccactgaggacctgaacctaactgaaaacatttctcaaggagatagaataagtgaaagaaaattggatttattgagcctcaaaaatatgagtgaagcacaatcaaagaatgaatttctttcaagagaactaattgaaaaagaaagagatttagaaaggagtaggacagtgatagccaaatttcagaataaattaaaagaattagttgaagaaaataagcaacttgaagaaggtatgaaagaaatattgcaagcaattaaggaaatgcagaaagatcctgatgttaaaggaggagaaacatctctaattatccctagccttgaaagactagttaatgctatagaatcaaagaatgcagaaggaatctttgatgcgagtctgcatttgaaagcccaagttgatcagcttaccggaagaaatgaagaattaagacaggagctcagggaatctcggaaagaggctataaattattcacagcagttggcaaaagctaatttaaagatagaccatcttgaaaaagaaactagtcttttacgacaatcagaaggatcgaatgttgtttttaaaggaattgacttacctgatgggatagcaccatctagtgccagtatcattaattctcagaatgaatatttaatacatttgttacaggaactagaaaataaagaaaaaaagttaaagaatttagaagattctcttgaagattacaacagaaaatttgctgtaattcgtcatcaacaaagtttgttgtataaagaatacctaagtgaaaaggagacctggaaaacagaatctaaaacaataaaagaggaaaagagaaaacttgaggatcaagtccaacaagatgctataaaagtaaaagaatataataatttgctcaatgctcttcagatggattcggatgaaatgaaaaaaatacttgca

SEQ ID NO: 22 - DNA, 3090 bp, Homo sapiens
gagtccctcagaatgcaactgctagactatcaggcacagtctgatgaaaagtcgctcattgccaagttgcaccaacataatgtctctcttcaactgagtgaggctactgctcttggtaagttggagtcaattacatctaaactgcagaagatggaggcctacaacttgcgcttagagcagaaacttgatgaaaaagaacaggctctctattatgctcgtttggagggaagaaacagagcaaaacatctgcgccaaacaattcagtctctacgacgacagtttagtggagctttacccttggcacaacaggaaaagttctccaaaacaatgattcaactacaaaatgacaaacttaagataatgcaagaaatgaaaaattctcaacaagaacatagaaatatggagaacaaaacattggagatggaattaaaattaaagggcctggaagagttaataagcactttaaaggataccaaaggagcccaaaaggtaatcaactggcatatgaaaatagaagaacttcgtcttcaagaacttaaactaaatcgggaattagtcaaggataaagaagaaataaaatatttgaataacataatttctgaatatgaacgtacaatcagcagtcttgaagaagaaattgtgcaacagaacaagtttcatgaagaaagacaaatggcctgggatcaaagagaagttgacctggaacgccaactagacatttttgaccgtcagcaaaatgaaatactaaatgcggcacaaaagtttgaagaagctacaggatcaatccctgaccctagtttgccccttccaaatcaacttgagatcgctctaaggaaaattaaggagaacattcgaataattctagaaacacgggcaacttgcaaatcactagaagagaaactaaaagagaaagaatctgctttaaggttagcagaacaaaatatactgtcaagagacaaagtaatcaatgaactgaggcttcgattgcctgccactgcagaaagagaaaagctcatagctgagctaggcagaaaagagatggaaccaaaatctcaccacacattgaaaattgctcatcaaaccattgcaaacatgcaagcaaggttaaatcaaaaagaagaagtattaaagaagtatcaacgtcttctagaaaaagccagagaggagcaaagagaaattgtgaagaaacatgaggaagaccttcatattcttcatcacagattagaactacaggctgatagttcactaaataaattcaaacaaacggcttgggatttaatgaaacagtctcccactccagttcctaccaacaagcattttattcgtctggctgagatggaacagacagtagcagaacaagatgactctctttcctcactcttggtcaaactaaagaaagtatcacaagatttggagagacaaagagaaatcactgaattaaaagtaaaagaatttgaaaatatcaaattacagcttcaagaaaaccatgaagatgaagtgaaaaaagtaaaagcggaagtagaggatttaaagtatcttctggacacaactggcatgactgttgatcaggttttgggaatacgagctttggagtcagaaaaagaattggaagaattaaaaaagagaaatcttgacttagaaaatgatatattgtatatgagggcccaccaagctcttcctcgagattctgttgtagaagatttacatttacaaaatagatacctccaagaaaaacttcatgctttagaaaaacagttttcaaaggatacatattctaagccttcaatttcaggaatagagtcagatgatcattgtcagagagaacaggagcttcagaaggaaaacttgaagttgtcatctgaaaatattgaactgaaatttcagcttgaacaagcaaataaagatttgccaagattaaagaatcaagtcagagatttgaaggaaatgtgtgaatttcttaagaaagaaaaagcagaagttcagcggaaacttggccatgttagagggtctggtagaagtggaaagacaatcccagaactggaaaaaaccattggtttaatgaaaaaagtagttgaaaaagtccagagagaaaatgaacagttgaaaaaagcatcaggaatattgactagtgaaaaaatggctaatattgagcaggaaaatgaaaaattgaaggctgaattagaaaaacttaaagctcatcttgggcatcagttgagcatgcactatgaatccaagaccaaaggcacagaaaaaattattgctgaaaatgaaaggcttcgtaaagaacttaaaaaagaaactgatgctgcagagaaattacggatagcaaagaataatttagagatattaaatgagaagatgacagttcaactagaagagactggtaagagattgcagtttgcagaaagcagaggtccacagcttgaaggtgctgacagtaagagctggaaatccattgtggttacaagaatgtatgaaaccaagttaaaagaattggaaactgatattgccaaaaaaaatcaaagcattactgaccttaaacagcttgtaaaagaagcaacagagagagaacaaaaagttaacaaatacaatgaagaccttgaacaacagattaagattcttaaacatgttcctgaaggtgctgagacagagcaaggccttaaacgggagcttcaagttcttagattagctaatcatcagctggataaagagaaagcagaattaatccatcagatagaagctaacaaggaccaaagtggagctgaaagcaccatacctgatgctgatcaactaaaggaaaaaataaaagatctagagacacagctcaaaatgtcagatctagaaaagcagcatttgaaggaggaaataaagaagctgaaaaaagaactggaaaattttgatccttcattttttgaagaaattgaagatcttaagtataattacaaggaagaagtgaagaagaatattctcttagaagagaaggtaaaaaaactttcagaacaattgggagttgaattaactagccctgttgctgcttctgaagagtttgaagatgaagaagaaagtcctgttaatttccccatttactaa

SEQ ID NO: 23 - DNA, 3846 bp, Homo sapiens
actgaaaacatttctcaaggagatagaataagtgaaagaaaattggatttattgagcctcaaaaatatgagtgaagcacaatcaaagaatgaatttctttcaagagaactaattgaaaaagaaagagatttagaaaggagtaggacagtgatagccaaatttcagaataaattaaaagaattagttgaagaaaataagcaacttgaagaaggtatgaaagaaatattgcaagcaattaaggaaatgcagaaagatcctgatgttaaaggaggagaaacatctctaattatccctagccttgaaagactagttaatgctatagaatcaaagaatgcagaaggaatctttgatgcgagtctgcatttgaaagcccaagttgatcagcttaccggaagaaatgaagaattaagacaggagctcagggaatctcggaaagaggctataaattattcacagcagttggcaaaagctaatttaaagatagaccatcttgaaaaagaaactagtcttttacgacaatcagaaggatcgaatgttgtttttaaaggaattgacttacctgatgggatagcaccatctagtgccagtatcattaattctcagaatgaatatttaatacatttgttacaggaactagaaaataaagaaaaaaagttaaagaatttagaagattctcttgaagattacaacagaaaatttgctgtaattcgtcatcaacaaagtttgttgtataaagaatacctaagtgaaaaggagacctggaaaacagaatctaaaacaataaaagaggaaaagagaaaacttgaggatcaagtccaacaagatgctataaaagtaaaagaatataataatttgctcaatgctcttcagatggattcggatgaaatgaaaaaaatacttgcagaaaatagtaggaaaattactgttttgcaagtgaatgaaaaatcacttataaggcaatatacaaccttagtagaattggagcgacaacttagaaaagaaaatgagaagcaaaagaatgaattgttgtcaatggaggctgaagtttgtgaaaaaattgggtgtttgcaaagatttaaggaaatggccattttcaagattgcagctctccaaaaagttgtagataatagtgtttctttgtctgaactagaactggctaataaacagtacaatgaactgactgctaagtacagggacatcttgcaaaaagataatatgcttgttcaaagaacaagtaacttggaacacctggagtgtgaaaacatctccttaaaagaacaagtggagtctataaataaagaactggagattaccaaggaaaaacttcacactattgaacaagcctgggaacaggaaactaaattaggtaatgaatctagcatggataaggcaaagaaatcaataaccaacagtgacattgtttccatttcaaaaaaaataactatgctggaaatgaaggaattaaatgaaaggcagcgggctgaacattgtcaaaaaatgtatgaacacttacggacttcgttaaagcaaatggaggaacgtaattttgaattggaaaccaaatttgctgagcttaccaaaatcaatttggatgcacagaaggtggaacagatgttaagagatgaattagctgatagtgtgagcaaggcagtaagtgatgctgataggcaacggattctagaattagagaagaatgaaatggaactaaaagttgaagtgtcaaaactgagagagatttctgatattgccagaagacaagttgaaattttgaatgcacaacaacaatctagggacaaggaagtaaaattgaaagaagcacttaaaacaagtaaaaacagagaaaactcactaactgataatttgaatgacttaaataatgaactgcaaaagaaacaaaaagcctataataaaatacttagagagaaagaggaaattgatcaagagaatgatgaactgaaaaggcaaattaaaagactaaccagtggattacagggcaaacccctgacagataataaacaaagtctaattgaagaactccaaaggaaagttaaaaaactagagaaccaattagagggaaaggtggaggaagtagacctaaaacctatgaaagaaaagaatgctaaagaagaattaattaggtgggaagaaggtaaaaagtggcaagccaaaatagaaggaattcgaaacaagttaaaagagaaagagggggaagtctttactttaacaaagcagttgaatactttgaaggatctttttgccaaagccgataaagagaaacttactttgcagaggaaactaaaaacaactggcatgactgttgatcaggttttgggaatacgagctttggagtcagaaaaagaattggaagaattaaaaaagagaaatcttgacttagaaaatgatatattgtatatgagggcccaccaagctcttcctcgagattctgttgtagaagatttacatttacaaaatagatacctccaagaaaaacttcatgctttagaaaaacagttttcaaaggatacatattctaagccttcaatttcaggaatagagtcagatgatcattgtcagagagaacaggagcttcagaaggaaaacttgaagttgtcatctgaaaatattgaactgaaatttcagcttgaacaagcaaataaagatttgccaagattaaagaatcaagtcagagatttgaaggaaatgtgtgaatttcttaagaaagaaaaagcagaagttcagcggaaacttggccatgttagagggtctggtagaagtggaaagacaatcccagaactggaaaaaaccattggtttaatgaaaaaagtagttgaaaaagtccagagagaaaatgaacagttgaaaaaagcatcaggaatattgactagtgaaaaaatggctaatattgagcaggaaaatgaaaaattgaaggctgaattagaaaaacttaaagctcatcttgggcatcagttgagcatgcactatgaatccaagaccaaaggcacagaaaaaattattgctgaaaatgaaaggcttcgtaaagaacttaaaaaagaaactgatgctgcagagaaattacggatagcaaagaataatttagagatattaaatgagaagatgacagttcaactagaagagactggtaagagattgcagtttgcagaaagcagaggtccacagcttgaaggtgctgacagtaagagctggaaatccattgtggttacaagaatgtatgaaaccaagttaaaagaattggaaactgatattgccaaaaaaaatcaaagcattactgaccttaaacagcttgtaaaagaagcaacagagagagaacaaaaagttaacaaatacaatgaagaccttgaacaacagattaagattcttaaacatgttcctgaaggtgctgagacagagcaaggccttaaacgggagcttcaagttcttagattagctaatcatcagctggataaagagaaagcagaattaatccatcagatagaagctaacaaggaccaaagtggagctgaaagcaccatacctgatgctgatcaactaaaggaaaaaataaaagatctagagacacagctcaaaatgtcagatctagaaaagcagcatttgaaggaggaaataaagaagctgaaaaaagaactggaaaattttgatccttcattttttgaagaaattgaagatcttaagtataattacaaggaagaagtgaagaagaatattctcttagaagagaaggtaaaaaaactttcagaacaattgggagttgaattaactagccctgttgctgcttctgaagagtttgaagatgaagaagaaagtcctgttaatttccccatttactaa

SEQ ID NO: 24 - DNA, 2358 bp, Homo sapiens
gagtccctcagaatgcaactgctagactatcaggcacagtctgatgaaaagtcgctcattgccaagttgcaccaacataatgtctctcttcaactgagtgaggctactgctcttggtaagttggagtcaattacatctaaactgcagaagatggaggcctacaacttgcgcttagagcagaaacttgatgaaaaagaacaggctctctattatgctcgtttggagggaagaaacagagcaaaacatctgcgccaaacaattcagtctctacgacgacagtttagtggagctttacccttggcacaacaggaaaagttctccaaaacaatgattcaactacaaaatgacaaacttaagataatgcaagaaatgaaaaattctcaacaagaacatagaaatatggagaacaaaacattggagatggaattaaaattaaagggcctggaagagttaataagcactttaaaggataccaaaggagcccaaaaggtaatcaactggcatatgaaaatagaagaacttcgtcttcaagaacttaaactaaatcgggaattagtcaaggataaagaagaaataaaatatttgaataacataatttctgaatatgaacgtacaatcagcagtcttgaagaagaaattgtgcaacagaacaagtttcatgaagaaagacaaatggcctgggatcaaagagaagttgacctggaacgccaactagacatttttgaccgtcagcaaaatgaaatactaaatgcggcacaaaagtttgaagaagctacaggatcaatccctgaccctagtttgccccttccaaatcaacttgagatcgctctaaggaaaattaaggagaacattcgaataattctagaaacacgggcaacttgcaaatcactagaagagaaactaaaagagaaagaatctgctttaaggttagcagaacaaaatatactgtcaagagacaaagtaatcaatgaactgaggcttcgattgcctgccactgcagaaagagaaaagctcatagctgagctaggcagaaaagagatggaaccaaaatctcaccacacattgaaaattgctcatcaaaccattgcaaacatgcaagcaaggttaaatcaaaaagaagaagtattaaagaagtatcaacgtcttctagaaaaagccagagaggagcaaagagaaattgtgaagaaacatgaggaagaccttcatattcttcatcacagattagaactacaggctgatagttcactaaataaattcaaacaaacggcttgggatttaatgaaacagtctcccactccagttcctaccaacaagcattttattcgtctggctgagatggaacagacagtagcagaacaagatgactctctttcctcactcttggtcaaactaaagaaagtatcacaagatttggagagacaaagagaaatcactgaattaaaagtaaaagaatttgaaaatatcaaattacagcttcaagaaaaccatgaagatgaagtgaaaaaagtaaaagcggaagtagaggatttaaagtatcttctggaccagtcacaaaaggagtcacagtgtttaaaatctgaacttcaggctcaaaaagaagcaaattcaagagctccaacaactacaatgagaaatctagtagaacggctaaagagccaattagccttgaaggagaaacaacagaaagcacttagtcgggcacttttagaactccgggcagaaatgacagcagctgctgaagaacgtattatttctgcaacttctcaaaaagaggcccatctcaatgttcaacaaatcgttgatcgacatactagagagctaaagacacaagttgaagatttaaatgaaaatcttttaaaattgaaagaagcacttaaaacaagtaaaaacagagaaaactcactaactgataatttgaatgacttaaataatgaactgcaaaagaaacaaaaagcctataataaaatacttagagagaaagaggaaattgatcaagagaatgatgaactgaaaaggcaaattaaaagactaaccagtggattacagggcaaacccctgacagataataaacaaagtctaattgaagaactccaaaggaaagttaaaaaactagagaaccaattagagggaaaggtggaggaagtagacctaaaacctatgaaagaaaagaatgctaaagaagaattaattaggtgggaagaaggtaaaaagtggcaagccaaaatagaaggaattcgaaacaagttaaaagagaaagagggggaagtctttactttaacaaagcagttgaatactttgaaggatctttttgccaaagccgataaagagaaacttactttgcagaggaaactaaaaaca

SEQ ID NO: 25 - DNA, 2745 bp, Homo sapiens
atattaacaaaggaaatcaataaacttgaattgaagatcagtgatttccttgatgaaaatgaggcacttagagagcgtgtgggccttgaaccaaagacaatgattgatttaactgaatttagaaatagcaaacacttaaaacagcagcagtacagagctgaaaaccagattcttttgaaagagattgaaagtctagaggaagaacgacttgatctgaaaaaaaaaattcgtcaaatggctcaagaaagaggaaaaagaagtgcaacttcaggattaaccactgaggacctgaacctaactgaaaacatttctcaaggagatagaataagtgaaagaaaattggatttattgagcctcaaaaatatgagtgaagcacaatcaaagaatgaatttctttcaagagaactaattgaaaaagaaagagatttagaaaggagtaggacagtgatagccaaatttcagaataaattaaaagaattagttgaagaaaataagcaacttgaagaaggtatgaaagaaatattgcaagcaattaaggaaatgcagaaagatcctgatgttaaaggaggagaaacatctctaattatccctagccttgaaagactagttaatgctatagaatcaaagaatgcagaaggaatctttgatgcgagtctgcatttgaaagcccaagttgatcagcttaccggaagaaatgaagaattaagacaggagctcagggaatctcggaaagaggctataaattattcacagcagttggcaaaagctaatttaaagatagaccatcttgaaaaagaaactagtcttttacgacaatcagaaggatcgaatgttgtttttaaaggaattgacttacctgatgggatagcaccatctagtgccagtatcattaattctcagaatgaatatttaatacatttgttacaggaactagaaaataaagaaaaaaagttaaagaatttagaagattctcttgaagattacaacagaaaatttgctgtaattcgtcatcaacaaagtttgttgtataaagaatacctaagtgaaaaggagacctggaaaacagaatctaaaacaataaaagaggaaaagagaaaacttgaggatcaagtccaacaagatgctataaaagtaaaagaatataataatttgctcaatgctcttcagatggattcggatgaaatgaaaaaaatacttgcaacaactggcatgactgttgatcaggttttgggaatacgagctttggagtcagaaaaagaattggaagaattaaaaaagagaaatcttgacttagaaaatgatatattgtatatgagggcccaccaagctcttcctcgagattctgttgtagaagatttacatttacaaaatagatacctccaagaaaaacttcatgctttagaaaaacagttttcaaaggatacatattctaagccttcaatttcaggaatagagtcagatgatcattgtcagagagaacaggagcttcagaaggaaaacttgaagttgtcatctgaaaatattgaactgaaatttcagcttgaacaagcaaataaagatttgccaagattaaagaatcaagtcagagatttgaaggaaatgtgtgaatttcttaagaaagaaaaagcagaagttcagcggaaacttggccatgttagagggtctggtagaagtggaaagacaatcccagaactggaaaaaaccattggtttaatgaaaaaagtagttgaaaaagtccagagagaaaatgaacagttgaaaaaagcatcaggaatattgactagtgaaaaaatggctaatattgagcaggaaaatgaaaaattgaaggctgaattagaaaaacttaaagctcatcttgggcatcagttgagcatgcactatgaatccaagaccaaaggcacagaaaaaattattgctgaaaatgaaaggcttcgtaaagaacttaaaaaagaaactgatgctgcagagaaattacggatagcaaagaataatttagagatattaaatgagaagatgacagttcaactagaagagactggtaagagattgcagtttgcagaaagcagaggtccacagcttgaaggtgctgacagtaagagctggaaatccattgtggttacaagaatgtatgaaaccaagttaaaagaattggaaactgatattgccaaaaaaaatcaaagcattactgaccttaaacagcttgtaaaagaagcaacagagagagaacaaaaagttaacaaatacaatgaagaccttgaacaacagattaagattcttaaacatgttcctgaaggtgctgagacagagcaaggccttaaacgggagcttcaagttcttagattagctaatcatcagctggataaagagaaagcagaattaatccatcagatagaagctaacaaggaccaaagtggagctgaaagcaccatacctgatgctgatcaactaaaggaaaaaataaaagatctagagacacagctcaaaatgtcagatctagaaaagcagcatttgaaggaggaaataaagaagctgaaaaaagaactggaaaattttgatccttcattttttgaagaaattgaagatcttaagtataattacaaggaagaagtgaagaagaatattctcttagaagagaaggtaaaaaaactttcagaacaattgggagttgaattaactagccctgttgctgcttctgaagagtttgaagatgaagaagaaagtcctgttaatttccccatttactaa

SEQ ID NO: 26 - DNA, 2655 bp, Homo sapiens
atattaacaaaggaaatcaataaacttgaattgaagatcagtgatttccttgatgaaaatgaggcacttagagagcgtgtgggccttgaaccaaagacaatgattgatttaactgaatttagaaatagcaaacacttaaaacagcagcagtacagagctgaaaaccagattcttttgaaagagattgaaagtctagaggaagaacgacttgatctgaaaaaaaaaattcgtcaaatggctcaagaaagaggaaaaagaagtgcaacttcaggattaaccactgaggacctgaacctagagtccctcagaatgcaactgctagactatcaggcacagtctgatgaaaagtcgctcattgccaagttgcaccaacataatgtctctcttcaactgagtgaggctactgctcttggtaagttggagtcaattacatctaaactgcagaagatggaggcctacaacttgcgcttagagcagaaacttgatgaaaaagaacaggctctctattatgctcgtttggagggaagaaacagagcaaaacatctgcgccaaacaattcagtctctacgacgacagtttagtggagctttacccttggcacaacaggaaaagttctccaaaacaatgattcaactacaaaatgacaaacttaagataatgcaagaaatgaaaaattctcaacaagaacatagaaatatggagaacaaaacattggagatggaattaaaattaaagggcctggaagagttaataagcactttaaaggataccaaaggagcccaaaaggtaatcaactggcatatgaaaatagaagaacttcgtcttcaagaacttaaactaaatcgggaattagtcaaggataaagaagaaataaaatatttgaataacataatttctgaatatgaacgtacaatcagcagtcttgaagaagaaattgtgcaacagaacaagtttcatgaagaaagacaaatggcctgggatcaaagagaagttgacctggaacgccaactagacatttttgaccgtcagcaaaatgaaatactaaatgcggcacaaaagtttgaagaagctacaggatcaatccctgaccctagtttgccccttccaaatcaacttgagatcgctctaaggaaaattaaggagaacattcgaataattctagaaacacgggcaacttgcaaatcactagaagagaaactaaaagagaaagaatctgctttaaggttagcagaacaaaatatactgtcaagagacaaagtaatcaatgaactgaggcttcgattgcctgccactgcagaaagagaaaagctcatagctgagctaggcagaaaagagatggaaccaaaatctcaccacacattgaaaattgctcatcaaaccattgcaaacatgcaagcaaggttaaatcaaaaagaagaagtattaaagaagtatcaacgtcttctagaaaaagccagagaggagcaaagagaaattgtgaagaaacatgaggaagaccttcatattcttcatcacagattagaactacaggctgatagttcactaaataaattcaaacaaacggcttgggatttaatgaaacagtctcccactccagttcctaccaacaagcattttattcgtctggctgagatggaacagacagtagcagaacaagatgactctctttcctcactcttggtcaaactaaagaaagtatcacaagatttggagagacaaagagaaatcactgaattaaaagtaaaagaatttgaaaatatcaaattacagcttcaagaaaaccatgaagatgaagtgaaaaaagtaaaagcggaagtagaggatttaaagtatcttctggaccagtcacaaaaggagtcacagtgtttaaaatctgaacttcaggctcaaaaagaagcaaattcaagagctccaacaactacaatgagaaatctagtagaacggctaaagagccaattagccttgaaggagaaacaacagaaagcacttagtcgggcacttttagaactccgggcagaaatgacagcagctgctgaagaacgtattatttctgcaacttctcaaaaagaggcccatctcaatgttcaacaaatcgttgatcgacatactagagagctaaagacacaagttgaagatttaaatgaaaatcttttaaaattgaaagaagcacttaaaacaagtaaaaacagagaaaactcactaactgataatttgaatgacttaaataatgaactgcaaaagaaacaaaaagcctataataaaatacttagagagaaagaggaaattgatcaagagaatgatgaactgaaaaggcaaattaaaagactaaccagtggattacagggcaaacccctgacagataataaacaaagtctaattgaagaactccaaaggaaagttaaaaaactagagaaccaattagagggaaaggtggaggaagtagacctaaaacctatgaaagaaaagaatgctaaagaagaattaattaggtgggaagaaggtaaaaagtggcaagccaaaatagaaggaattcgaaacaagttaaaagagaaagagggggaagtctttactttaacaaagcagttgaatactttgaaggatctttttgccaaagccgataaagagaaacttactttgcagaggaaactaaaaaca

SEQ ID NO: 27 - DNA, 2013 bp, Homo sapiens
atattaacaaaggaaatcaataaacttgaattgaagatcagtgatttccttgatgaaaatgaggcacttagagagcgtgtgggccttgaaccaaagacaatgattgatttaactgaatttagaaatagcaaacacttaaaacagcagcagtacagagctgaaaaccagattcttttgaaagagattgaaagtctagaggaagaacgacttgatctgaaaaaaaaaattcgtcaaatggctcaagaaagaggaaaaagaagtgcaacttcaggattaaccactgaggacctgaacctaactgaaaacatttctcaaggagatagaataagtgaaagaaaattggatttattgagcctcaaaaatatgagtgaagcacaatcaaagaatgaatttctttcaagagaactaattgaaaaagaaagagatttagaaaggagtaggacagtgatagccaaatttcagaataaattaaaagaattagttgaagaaaataagcaacttgaagaaggtatgaaagaaatattgcaagcaattaaggaaatgcagaaagatcctgatgttaaaggaggagaaacatctctaattatccctagccttgaaagactagttaatgctatagaatcaaagaatgcagaaggaatctttgatgcgagtctgcatttgaaagcccaagttgatcagcttaccggaagaaatgaagaattaagacaggagctcagggaatctcggaaagaggctataaattattcacagcagttggcaaaagctaatttaaagatagaccatcttgaaaaagaaactagtcttttacgacaatcagaaggatcgaatgttgtttttaaaggaattgacttacctgatgggatagcaccatctagtgccagtatcattaattctcagaatgaatatttaatacatttgttacaggaactagaaaataaagaaaaaaagttaaagaatttagaagattctcttgaagattacaacagaaaatttgctgtaattcgtcatcaacaaagtttgttgtataaagaatacctaagtgaaaaggagacctggaaaacagaatctaaaacaataaaagaggaaaagagaaaacttgaggatcaagtccaacaagatgctataaaagtaaaagaatataataatttgctcaatgctcttcagatggattcggatgaaatgaaaaaaatacttgcacagtcacaaaaggagtcacagtgtttaaaatctgaacttcaggctcaaaaagaagcaaattcaagagctccaacaactacaatgagaaatctagtagaacggctaaagagccaattagccttgaaggagaaacaacagaaagcacttagtcgggcacttttagaactccgggcagaaatgacagcagctgctgaagaacgtattatttctgcaacttctcaaaaagaggcccatctcaatgttcaacaaatcgttgatcgacatactagagagctaaagacacaagttgaagatttaaatgaaaatcttttaaaattgaaagaagcacttaaaacaagtaaaaacagagaaaactcactaactgataatttgaatgacttaaataatgaactgcaaaagaaacaaaaagcctataataaaatacttagagagaaagaggaaattgatcaagagaatgatgaactgaaaaggcaaattaaaagactaaccagtggattacagggcaaacccctgacagataataaacaaagtctaattgaagaactccaaaggaaagttaaaaaactagagaaccaattagagggaaaggtggaggaagtagacctaaaacctatgaaagaaaagaatgctaaagaagaattaattaggtgggaagaaggtaaaaagtggcaagccaaaatagaaggaattcgaaacaagttaaaagagaaagagggggaagtctttactttaacaaagcagttgaatactttgaaggatctttttgccaaagccgataaagagaaacttactttgcagaggaaactaaaaaca

SEQ ID NO: 28 - DNA, 1716 bp, Homo sapiens
actgaaaacatttctcaaggagatagaataagtgaaagaaaattggatttattgagcctcaaaaatatgagtgaagcacaatcaaagaatgaatttctttcaagagaactaattgaaaaagaaagagatttagaaaggagtaggacagtgatagccaaatttcagaataaattaaaagaattagttgaagaaaataagcaacttgaagaaggtatgaaagaaatattgcaagcaattaaggaaatgcagaaagatcctgatgttaaaggaggagaaacatctctaattatccctagccttgaaagactagttaatgctatagaatcaaagaatgcagaaggaatctttgatgcgagtctgcatttgaaagcccaagttgatcagcttaccggaagaaatgaagaattaagacaggagctcagggaatctcggaaagaggctataaattattcacagcagttggcaaaagctaatttaaagatagaccatcttgaaaaagaaactagtcttttacgacaatcagaaggatcgaatgttgtttttaaaggaattgacttacctgatgggatagcaccatctagtgccagtatcattaattctcagaatgaatatttaatacatttgttacaggaactagaaaataaagaaaaaaagttaaagaatttagaagattctcttgaagattacaacagaaaatttgctgtaattcgtcatcaacaaagtttgttgtataaagaatacctaagtgaaaaggagacctggaaaacagaatctaaaacaataaaagaggaaaagagaaaacttgaggatcaagtccaacaagatgctataaaagtaaaagaatataataatttgctcaatgctcttcagatggattcggatgaaatgaaaaaaatacttgcacagtcacaaaaggagtcacagtgtttaaaatctgaacttcaggctcaaaaagaagcaaattcaagagctccaacaactacaatgagaaatctagtagaacggctaaagagccaattagccttgaaggagaaacaacagaaagcacttagtcgggcacttttagaactccgggcagaaatgacagcagctgctgaagaacgtattatttctgcaacttctcaaaaagaggcccatctcaatgttcaacaaatcgttgatcgacatactagagagctaaagacacaagttgaagatttaaatgaaaatcttttaaaattgaaagaagcacttaaaacaagtaaaaacagagaaaactcactaactgataatttgaatgacttaaataatgaactgcaaaagaaacaaaaagcctataataaaatacttagagagaaagaggaaattgatcaagagaatgatgaactgaaaaggcaaattaaaagactaaccagtggattacagggcaaacccctgacagataataaacaaagtctaattgaagaactccaaaggaaagttaaaaaactagagaaccaattagagggaaaggtggaggaagtagacctaaaacctatgaaagaaaagaatgctaaagaagaattaattaggtgggaagaaggtaaaaagtggcaagccaaaatagaaggaattcgaaacaagttaaaagagaaagagggggaagtctttactttaacaaagcagttgaatactttgaaggatctttttgccaaagccgataaagagaaacttactttgcagaggaaactaaaaaca

SEQ ID NO: 29 - DNA, 2406 bp, Homo sapiens
atgccacctaatataaactggaaagaaataatgaaagttgacccagatgacctgccccgtcaagaagaactggcagataatttattgatttccttatccaaggtggaagtaaatgagctaaaaagtgaaaagcaagaaaatgtgatacaccttttcagaattactcagtcactaatgaagatgaaagctcaagaagtggagctggctttggaagaagtagaaaaagctggagaagaacaagcaaaatttgaaaatcaattaaaaactaaagtaatgaaactggaaaatgaactggagatggctcagcagtctgcaggtggacgagatactcggtttttacgtaatgaaatttgccaacttgaaaaacaattagaacaaaaagatagagaattggaggacatggaaaaggagttggagaaagagaagaaagttaatgagcaattggctcttcgaaatgaggaggcagaaaatgaaaacagcaaattaagaagagagaacaaacgtctaaagaaaaagaatgaacaactttgtcaggatattattgactaccagaaacaaatagattcacagaaagaaacacttttatcaagaagaggggaaactgaaaacatttctcaaggagatagaataagtgaaagaaaattggatttattgagcctcaaaaatatgagtgaagcacaatcaaagaatgaatttctttcaagagaactaattgaaaaagaaagagatttagaaaggagtaggacagtgatagccaaatttcagaataaattaaaagaattagttgaagaaaataagcaacttgaagaaggtatgaaagaaatattgcaagcaattaaggaaatgcagaaagatcctgatgttaaaggaggagaaacatctctaattatccctagccttgaaagactagttaatgctatagaatcaaagaatgcagaaggaatctttgatgcgagtctgcatttgaaagcccaagttgatcagcttaccggaagaaatgaagaattaagacaggagctcagggaatctcggaaagaggctataaattattcacagcagttggcaaaagctaatttaaagatagaccatcttgaaaaagaaactagtcttttacgacaatcagaaggatcgaatgttgtttttaaaggaattgacttacctgatgggatagcaccatctagtgccagtatcattaattctcagaatgaatatttaatacatttgttacaggaactagaaaataaagaaaaaaagttaaagaatttagaagattctcttgaagattacaacagaaaatttgctgtaattcgtcatcaacaaagtttgttgtataaagaatacctaagtgaaaaggagacctggaaaacagaatctaaaacaataaaagaggaaaagagaaaacttgaggatcaagtccaacaagatgctataaaagtaaaagaatataataatttgctcaatgctcttcagatggattcggatgaaatgaaaaaaatacttgcagaaaatagtaggaaaattactgttttgcaagtgaatgaaaaatcacttataaggcaatatacaaccttagtagaattggagcgacaacttagaaaagaaaatgagaagcaaaagaatgaattgttgtcaatggaggctgaagtttgtgaaaaaattgggtgtttgcaaagatttaaggaaatggccattttcaagattgcagctctccaaaaagttgtagataatagtgtttctttgtctgaactagaactggctaataaacagtacaatgaactgactgctaagtacagggacatcttgcaaaaagataatatgcttgttcaaagaacaagtaacttggaacacctggagtgtgaaaacatctccttaaaagaacaagtggagtctataaataaagaactggagattaccaaggaaaaacttcacactattgaacaagcctgggaacaggaaactaaattaggtaatgaatctagcatggataaggcaaagaaatcaataaccaacagtgacattgtttccatttcaaaaaaaataactatgctggaaatgaaggaattaaatgaaaggcagcgggctgaacattgtcaaaaaatgtatgaacacttacggacttcgttaaagcaaatggaggaacgtaattttgaattggaaaccaaatttgctgagcttaccaaaatcaatttggatgcacagaaggtggaacagatgttaagagatgaattagctgatagtgtgagcaaggcagtaagtgatgctgataggcaacggattctagaattagagaagaatgaaatggaactaaaagttgaagtgtcaaaactgagagagatttctgatattgccagaagacaagttgaaattttgaatgcacaacaacaatctagggacaaggaagtataa

SEQ ID NO: 30 - protein, 1316 aa, Homo sapiens
KNTCIIEDLKNELQRNKGASTLSQQTHMKIQSTLDILKEKTKEAERTAELAEADAREKDKELVEALKRLKDYESGVYGLEDAVVEIKNCKNQIKIRDREIEILTKEINKLELKISDFLDENEALRERVGLEPKTMIDLTEFRNSKHLKQQQYRAENQILLKEIESLEEERLDLKKKIRQMAQERGKRSATSGLTTEDLNLTENISQGDRISERKLDLLSLKNMSEAQSKNEFLSRELIEKERDLERSRTVIAKFQNKLKELVEENKQLEEGMKEILQAIKEMQKDPDVKGGETSLIIPSLERLVNAIESKNAEGIFDASLHLKAQVDQLTGRNEELRQELRESRKEAINYSQQLAKANLKIDHLEKETSLLRQSEGSNVVFKGIDLPDGIAPSSASIINSQNEYLIHLLQELENKEKKLKNLEDSLEDYNRKFAVIRHQQSLLYKEYLSEKETWKTESKTIKEEKRKLEDQVQQDAIKVKEYNNLLNALQMDSDEMKKILAENSRKITVLQVNEKSLIRQYTTLVELERQLRKENEKQKNELLSMEAEVCEKIGCLQRFKEMAIFKIAALQKVVDNSVSLSELELANKQYNELTAKYRDILQKDNMLVQRTSNLEHLECENISLKEQVESINKELEITKEKLHTIEQAWEQETKLGNESSMDKAKKSITNSDIVSISKKITMLEMKELNERQRAEHCQKMYEHLRTSLKQMEERNFELETKFAELTKINLDAQKVEQMLRDELADSVSKAVSDADRQRILELEKNEMELKVEVSKLREISDIARRQVEILNAQQQSRDKEVESLRMQLLDYQAQSDEKSLIAKLHQHNVSLQLSEATALGKLESITSKLQKMEAYNLRLEQKLDEKEQALYYARLEGRNRAKHLRQTIQSLRRQFSGALPLAQQEKFSKTMIQLQNDKLKIMQEMKNSQQEHRNMENKTLEMELKLKGLEELISTLKDTKGAQKVINWHMKIEELRLQELKLNRELVKDKEEIKYLNNIISEYERTISSLEEEIVQQNKFHEERQMAWDQREVDLERQLDIFDRQQNEILNAAQKFEEATGSIPDPSLPLPNQLEIALRKIKENIRIILETRATCKSLEEKLKEKESALRLAEQNILSRDKVINELRLRLPATAEREKLIAELGRKEMEPKSHHTLKIAHQTIANMQARLNQKEEVLKKYQRLLEKAREEQREIVKKHEEDLHILHHRLELQADSSLNKFKQTAWDLMKQSPTPVPTNKHFIRLAEMEQTVAEQDDSLSSLLVKLKKVSQDLERQREITELKVKEFENIKLQLQENHEDEVKKVKAEVEDLKYLLD

SEQ ID NO: 31 - protein, 514 aa, Homo sapiens
TTGMTVDQVLGIRALESEKELEELKKRNLDLENDILYMRAHQALPRDSVVEDLHLQNRYLQEKLHALEKQFSKDTYSKPSISGIESDDHCQREQELQKENLKLSSENIELKFQLEQANKDLPRLKNQVRDLKEMCEFLKKEKAEVQRKLGHVRGSGRSGKTIPELEKTIGLMKKVVEKVQRENEQLKKASGILTSEKMANIEQENEKLKAELEKLKAHLGHQLSMHYESKTKGTEKIIAENERLRKELKKETDAAEKLRIAKNNLEILNEKMTVQLEETGKRLQFAESRGPQLEGADSKSWKSIVVTRMYETKLKELETDIAKKNQSITDLKQLVKEATEREQKVNKYNEDLEQQIKILKHVPEGAETEQGLKRELQVLRLANHQLDKEKAELIHQIEANKDQSGAESTIPDADQLKEKIKDLETQLKMSDLEKQHLKEEIKKLKKELENFDPSFFEEIEDLKYNYKEEVKKNILLEEKVKKLSEQLGVELTSPVAASEEFEDEEESPVNFPIY

SEQ ID NO: 32 - DNA, 1545 bp, Homo sapiens
acaactggcatgactgttgatcaggttttgggaatacgagctttggagtcagaaaaagaattggaagaattaaaaaagagaaatcttgacttagaaaatgatatattgtatatgagggcccaccaagctcttcctcgagattctgttgtagaagatttacatttacaaaatagatacctccaagaaaaacttcatgctttagaaaaacagttttcaaaggatacatattctaagccttcaatttcaggaatagagtcagatgatcattgtcagagagaacaggagcttcagaaggaaaacttgaagttgtcatctgaaaatattgaactgaaatttcagcttgaacaagcaaataaagatttgccaagattaaagaatcaagtcagagatttgaaggaaatgtgtgaatttcttaagaaagaaaaagcagaagttcagcggaaacttggccatgttagagggtctggtagaagtggaaagacaatcccagaactggaaaaaaccattggtttaatgaaaaaagtagttgaaaaagtccagagagaaaatgaacagttgaaaaaagcatcaggaatattgactagtgaaaaaatggctaatattgagcaggaaaatgaaaaattgaaggctgaattagaaaaacttaaagctcatcttgggcatcagttgagcatgcactatgaatccaagaccaaaggcacagaaaaaattattgctgaaaatgaaaggcttcgtaaagaacttaaaaaagaaactgatgctgcagagaaattacggatagcaaagaataatttagagatattaaatgagaagatgacagttcaactagaagagactggtaagagattgcagtttgcagaaagcagaggtccacagcttgaaggtgctgacagtaagagctggaaatccattgtggttacaagaatgtatgaaaccaagttaaaagaattggaaactgatattgccaaaaaaaatcaaagcattactgaccttaaacagcttgtaaaagaagcaacagagagagaacaaaaagttaacaaatacaatgaagaccttgaacaacagattaagattcttaaacatgttcctgaaggtgctgagacagagcaaggccttaaacgggagcttcaagttcttagattagctaatcatcagctggataaagagaaagcagaattaatccatcagatagaagctaacaaggaccaaagtggagctgaaagcaccatacctgatgctgatcaactaaaggaaaaaataaaagatctagagacacagctcaaaatgtcagatctagaaaagcagcatttgaaggaggaaataaagaagctgaaaaaagaactggaaaattttgatccttcattttttgaagaaattgaagatcttaagtataattacaaggaagaagtgaagaagaatattctcttagaagagaaggtaaaaaaactttcagaacaattgggagttgaattaactagccctgttgctgcttctgaagagtttgaagatgaagaagaaagtcctgttaatttccccatttactaa

SEQ ID NO: 33 - DNA, 3948 bp, Homo sapiens
aagaatacttgtattattgaagatttgaaaaatgagctccaaagaaacaaaggtgcttcaaccctttctcaacagactcatatgaaaattcagtcaacgttagacattttaaaagagaaaactaaagaggctgagagaacagctgaactggctgaggctgatgctagggaaaaggataaagaattagttgaggctctgaagaggttaaaagattatgaatcgggagtatatggtttagaagatgctgtcgttgaaataaagaattgtaaaaaccaaattaaaataagagatcgagagattgaaatattaacaaaggaaatcaataaacttgaattgaagatcagtgatttccttgatgaaaatgaggcacttagagagcgtgtgggccttgaaccaaagacaatgattgatttaactgaatttagaaatagcaaacacttaaaacagcagcagtacagagctgaaaaccagattcttttgaaagagattgaaagtctagaggaagaacgacttgatctgaaaaaaaaaattcgtcaaatggctcaagaaagaggaaaaagaagtgcaacttcaggattaaccactgaggacctgaacctaactgaaaacatttctcaaggagatagaataagtgaaagaaaattggatttattgagcctcaaaaatatgagtgaagcacaatcaaagaatgaatttctttcaagagaactaattgaaaaagaaagagatttagaaaggagtaggacagtgatagccaaatttcagaataaattaaaagaattagttgaagaaaataagcaacttgaagaaggtatgaaagaaatattgcaagcaattaaggaaatgcagaaagatcctgatgttaaaggaggagaaacatctctaattatccctagccttgaaagactagttaatgctatagaatcaaagaatgcagaaggaatctttgatgcgagtctgcatttgaaagcccaagttgatcagcttaccggaagaaatgaagaattaagacaggagctcagggaatctcggaaagaggctataaattattcacagcagttggcaaaagctaatttaaagatagaccatcttgaaaaagaaactagtcttttacgacaatcagaaggatcgaatgttgtttttaaaggaattgacttacctgatgggatagcaccatctagtgccagtatcattaattctcagaatgaatatttaatacatttgttacaggaactagaaaataaagaaaaaaagttaaagaatttagaagattctcttgaagattacaacagaaaatttgctgtaattcgtcatcaacaaagtttgttgtataaagaatacctaagtgaaaaggagacctggaaaacagaatctaaaacaataaaagaggaaaagagaaaacttgaggatcaagtccaacaagatgctataaaagtaaaagaatataataatttgctcaatgctcttcagatggattcggatgaaatgaaaaaaatacttgcagaaaatagtaggaaaattactgttttgcaagtgaatgaaaaatcacttataaggcaatatacaaccttagtagaattggagcgacaacttagaaaagaaaatgagaagcaaaagaatgaattgttgtcaatggaggctgaagtttgtgaaaaaattgggtgtttgcaaagatttaaggaaatggccattttcaagattgcagctctccaaaaagttgtagataatagtgtttctttgtctgaactagaactggctaataaacagtacaatgaactgactgctaagtacagggacatcttgcaaaaagataatatgcttgttcaaagaacaagtaacttggaacacctggagtgtgaaaacatctccttaaaagaacaagtggagtctataaataaagaactggagattaccaaggaaaaacttcacactattgaacaagcctgggaacaggaaactaaattaggtaatgaatctagcatggataaggcaaagaaatcaataaccaacagtgacattgtttccatttcaaaaaaaataactatgctggaaatgaaggaattaaatgaaaggcagcgggctgaacattgtcaaaaaatgtatgaacacttacggacttcgttaaagcaaatggaggaacgtaattttgaattggaaaccaaatttgctgagcttaccaaaatcaatttggatgcacagaaggtggaacagatgttaagagatgaattagctgatagtgtgagcaaggcagtaagtgatgctgataggcaacggattctagaattagagaagaatgaaatggaactaaaagttgaagtgtcaaaactgagagagatttctgatattgccagaagacaagttgaaattttgaatgcacaacaacaatctagggacaaggaagtagagtccctcagaatgcaactgctagactatcaggcacagtctgatgaaaagtcgctcattgccaagttgcaccaacataatgtctctcttcaactgagtgaggctactgctcttggtaagttggagtcaattacatctaaactgcagaagatggaggcctacaacttgcgcttagagcagaaacttgatgaaaaagaacaggctctctattatgctcgtttggagggaagaaacagagcaaaacatctgcgccaaacaattcagtctctacgacgacagtttagtggagctttacccttggcacaacaggaaaagttctccaaaacaatgattcaactacaaaatgacaaacttaagataatgcaagaaatgaaaaattctcaacaagaacatagaaatatggagaacaaaacattggagatggaattaaaattaaagggcctggaagagttaataagcactttaaaggataccaaaggagcccaaaaggtaatcaactggcatatgaaaatagaagaacttcgtcttcaagaacttaaactaaatcgggaattagtcaaggataaagaagaaataaaatatttgaataacataatttctgaatatgaacgtacaatcagcagtcttgaagaagaaattgtgcaacagaacaagtttcatgaagaaagacaaatggcctgggatcaaagagaagttgacctggaacgccaactagacatttttgaccgtcagcaaaatgaaatactaaatgcggcacaaaagtttgaagaagctacaggatcaatccctgaccctagtttgccccttccaaatcaacttgagatcgctctaaggaaaattaaggagaacattcgaataattctagaaacacgggcaacttgcaaatcactagaagagaaactaaaagagaaagaatctgctttaaggttagcagaacaaaatatactgtcaagagacaaagtaatcaatgaactgaggcttcgattgcctgccactgcagaaagagaaaagctcatagctgagctaggcagaaaagagatggaaccaaaatctcaccacacattgaaaattgctcatcaaaccattgcaaacatgcaagcaaggttaaatcaaaaagaagaagtattaaagaagtatcaacgtcttctagaaaaagccagagaggagcaaagagaaattgtgaagaaacatgaggaagaccttcatattcttcatcacagattagaactacaggctgatagttcactaaataaattcaaacaaacggcttgggatttaatgaaacagtctcccactccagttcctaccaacaagcattttattcgtctggctgagatggaacagacagtagcagaacaagatgactctctttcctcactcttggtcaaactaaagaaagtatcacaagatttggagagacaaagagaaatcactgaattaaaagtaaaagaatttgaaaatatcaaattacagcttcaagaaaaccatgaagatgaagtgaaaaaagtaaaagcggaagtagaggatttaaagtatcttctggac

SEQ ID NO: 34 - DNA, 2406 bp, Homo sapiens; identical to SEQ ID NO: 29

SEQ ID NO: 35 - DNA, 2946 bp, Homo sapiens
atgcccccaaacatcaactggaaagagattatgaaagtggaccctgacgacctgcctagacaggaagaactggctgacaacctgctgatcagcctgtccaaggtggaagtgaatgagctgaagtctgagaagcaggagaacgtgatccacctgttcagaatcacccagagcctgatgaagatgaaggcacaggaggtggagctggccctggaggaggtggagaaggcaggagaggagcaggccaagttcgagaatcagctgaagaccaaagtgatgaagctggagaacgagctggagatggcacagcagtccgccggaggcagggatacacgctttctgcggaacgagatctgccagctggagaagcagctggagcagaaggacagggagctggaggatatggagaaggagctggagaaggagaagaaggtgaacgagcagctggccctgcgcaatgaggaggccgagaatgagaatagcaagctgcggagagagaacaagcggctgaagaagaagaacgagcagctgtgccaggacatcatcgattaccagaagcagatcgactcccagaaggagacactgctgagcaggaggggagaggactccgattatcgcagccagctgtccaagaagaattacgagctgatccagtatctggatgagatccagaccctgacagaggccaacgagaagatcgaggtgcagaaccaggagatgagaaagaatctggaggagtccgtgcaggagatggagaagatgaccgacgagtacaacaggatgaaggccatcgtgcaccagacagacaatgtgatcgatcagctgaagaaggagaacgaccactatcagctgcaggtgcaggagctgaccgatctgctgaagtccaagaatgaggaggacgatcccatcatggtggccgtgaacgccaaggtggaggagtggaagctgatcctgagctccaaggacgatgagatcatcgagtaccagcagatgctgcacaacctgcgcgagaagctgaagaatgcccagctggacgccgataagagcaatgtgatggcactgcagcagggaatccaggagagggactcccagatcaagatgctgaccgagcaggtggagcagtataccaaggagatggagaagacagagaacatctctcagggcgacagaatcagcgagaggaagctggatctgctgtccctgaagaacatgtccgaggcccagtctaagaatgagttcctgtcccgcgagctgatcgagaaggagcgggacctggagcggagccggacagtgatcgccaagtttcagaataagctgaaggagctggtggaggagaacaagcagctggaggagggcatgaaggagatcctgcaggccatcaaggagatgcagaaggacccagatgtgaagggcggcgagacaagcctgatcatcccctctctggagcgcctggtgaacgccatcgagagcaagaatgccgagggcatctttgacgcctccctgcacctgaaggcccaggtggatcagctgacaggccgcaatgaggagctgcggcaggagctgagagagtctaggaaggaggccatcaattacagccagcagctggccaaggccaacctgaagatcgaccacctggagaaggagacaagcctgctgcggcagtctgagggcagcaacgtggtgttcaagggaatcgacctgccagatggaatcgcaccttctagcgccagcatcatcaactcccagaatgagtacctgatccacctgctgcaggagctggagaacaaggagaagaagctgaagaatctggaggactctctggaggattataatagaaagtttgccgtgatcaggcaccagcagtccctgctgtacaaggagtatctgtctgagaaggagacatggaagacagagagcaagaccatcaaggaggagaagaggaagctggaggaccaggtgcagcaggatgccatcaaggtgaaggagtacaacaatctgctgaacgccctgcagatggactctgatgagatgaagaagatcctggccgagaatagcagaaagatcacagtgctgcaggtgaacgagaagtccctgatcaggcagtataccacactggtggagctggagcgccagctgcggaaggagaacgagaagcagaagaatgagctgctgtctatggaggccgaggtgtgcgagaagatcggctgtctgcagagattcaaggagatggccatctttaagatcgccgccctgcagaaggtggtggacaattctgtgagcctgtccgagctggagctggccaacaagcagtacaatgagctgaccgccaagtatcgcgacatcctgcagaaggataacatgctggtgcagcggacaagcaatctggagcacctggagtgcgagaacatcagcctgaaggagcaggtggagtccatcaacaaggagctggagatcaccaaggagaagctgcacacaatcgagcaggcctgggagcaggagacaaagctgggcaatgagtcctctatggacaaggccaagaagtctatcaccaacagcgatatcgtgtctatcagcaagaagatcacaatgctggagatgaaggagctgaatgagaggcagcgcgccgagcactgtcagaagatgtacgagcacctgagaacatccctgaagcagatggaggagaggaatttcgagctggagacaaagtttgccgagctgacaaagatcaacctggacgcccagaaggtggagcagatgctgagagacgagctggccgattccgtgtctaaggccgtgagcgacgccgatcggcagagaatcctggagctggagaagaacgagatggagctgaaggtggaggtgtccaagctgagggagatctctgatatcgctcggcggcaggtggagattctgaacgcacagcagcagtcacgggacaaggaagtctga

SEQ ID NO: 36 - protein, 981 aa, Homo sapiens
MPPNINWKEIMKVDPDDLPRQEELADNLLISLSKVEVNELKSEKQENVIHLFRITQSLMKMKAQEVELALEEVEKAGEEQAKFENQLKTKVMKLENELEMAQQSAGGRDTRFLRNEICQLEKQLEQKDRELEDMEKELEKEKKVNEQLALRNEEAENENSKLRRENKRLKKKNEQLCQDIIDYQKQIDSQKETLLSRRGEDSDYRSQLSKKNYELIQYLDEIQTLTEANEKIEVQNQEMRKNLEESVQEMEKMTDEYNRMKAIVHQTDNVIDQLKKENDHYQLQVQELTDLLKSKNEEDDPIMVAVNAKVEEWKLILSSKDDEIIEYQQMLHNLREKLKNAQLDADKSNVMALQQGIQERDSQIKMLTEQVEQYTKEMEKTENISQGDRISERKLDLLSLKNMSEAQSKNEFLSRELIEKERDLERSRTVIAKFQNKLKELVEENKQLEEGMKEILQAIKEMQKDPDVKGGETSLIIPSLERLVNAIESKNAEGIFDASLHLKAQVDQLTGRNEELRQELRESRKEAINYSQQLAKANLKIDHLEKETSLLRQSEGSNVVFKGIDLPDGIAPSSASIINSQNEYLIHLLQELENKEKKLKNLEDSLEDYNRKFAVIRHQQSLLYKEYLSEKETWKTESKTIKEEKRKLEDQVQQDAIKVKEYNNLLNALQMDSDEMKKILAENSRKITVLQVNEKSLIRQYTTLVELERQLRKENEKQKNELLSMEAEVCEKIGCLQRFKEMAIFKIAALQKVVDNSVSLSELELANKQYNELTAKYRDILQKDNMLVQRTSNLEHLECENISLKEQVESINKELEITKEKLHTIEQAWEQETKLGNESSMDKAKKSITNSDIVSISKKITMLEMKELNERQRAEHCQKMYEHLRTSLKQMEERNFELETKFAELTKINLDAQKVEQMLRDELADSVSKAVSDADRQRILELEKNEMELKVEVSKLREISDIARRQVEILNAQQQSRDKEV

SEQ ID NO: 37 - DNA, 973 bp, Gallus domesticus
gtgagcgggcgggacggcccttctcctccgggctgtaattagcgcttggtttaatgacggcttgtttcttttctgtggctgcgtgaaagccttgaggggctccgggagggccctttgtgcggggggagcggctcggggggtgcgtgcgtgtgtgtgtgcgtggggagcgccgcgtgcggctccgcgctgcccggcggctgtgagcgctgcgggcgcggcgcggggctttgtgcgctccgcagtgtgcgcgaggggagcgcggccgggggcggtgccccgcggtgcggggggggctgcgaggggaacaaaggctgcgtgcggggtgtgtgcgtgggggggtgagcagggggtgtgggcgcgtcggtcgggctgcaaccccccctgcacccccctccccgagttgctgagcacggcccggcttcgggtgcggggctccgtacggggcgtggcgcggggctcgccgtgccgggcggggggtggcggcaggtgggggtgccgggcggggcggggccgcctcgggccggggagggctcgggggaggggcgcggcggcccccggagcgccggcggctgtcgaggcgcggcgagccgcagccattgccttttatggtaatcgtgcgagagggcgcagggacttcctttgtcccaaatctgtgcggagccgaaatctgggaggcgccgccgcaccccctctagcgggcgcggggcgaagcggtgcggcgccggcaggaaggaaatgggcggggagggccttcgtgcgtcgccgcgccgccgtccccttctccctctccagcctcggggctgtccgcggggggacggctgccttcgggggggacggggcagggcggggttcggcttctggcgtgtgaccggcggctctagagcctctgctaaccatgttcatgccttcttctttttcctacagctcctgggcaacgtgctggttattgtgctgtctcatcattttggcaaag

SEQ ID NO: 38 - DNA, 172 bp, Artificial Sequence
  Synthetic Polynucleotide
gaactgaaaaaccagaaagttaactggtaagtttagtctttttgtcttttatttcaggtcccggatccggtggtggtgcaaatcaaagaactgctcctcagtggatgttgcctttacttctaggcctgtacggaagtgttacttctgctctaaaagctgcggaattgtaccc

SEQ ID NO: 39 - DNA, 384 bp, Unknown
  MBL intron
tcagatcgcctggagacgccatccacgctgttttgacctccatagaagacaccgggaccgatccagcctccgcggccgggaacggtgcattggaacgcggattccccgtgccaagagtgacgtaagtaccgcctatagagtctataggcccacccccttggcttcttatgcatgctatactgtttttggcttggggtctatacacccccgcttcctcatgtttgctgcccgtgaccagcacgtcaacgattttgtgggcacgggcgacaccgcagtgtagtctgagcagtactcgttgctgccgcgcgcgccaccagacataatagctgacagactaacagactgttcctttccatgggtcttttctgcagtcaccgtcgccgc